European Patent Application EP 4 729 620 A1, published April 22, 2026. Title: 用于治疗帕金森病的基因治疗载体及其用途. Applicant: 康霖生物科技（杭州）有限公司. The sequence listing filed with the application follows.

SEQUENCE LISTING (48 sequences)

SEQ ID NO: 1 - DNA, 814 bp, synthetic construct
  source 1..814: mol_type = other DNA
cgttacataacttacggtaaatggcccgcctggctgaccgcccaacgacccccgcccattgacgtcaataatgacgtatgttcccatagtaacgccaatagggactttccattgacgtcaatgggtggagtatttacggtaaactgcccacttggcagtacatcaagtgtatcatatgccaagtacgccccctattgacgtcaatgacggtaaatggcccgcctggcattatgcccagtacatgaccttatgggactttcctacttggcagtacatctacgtattagtcatcgctattaccatggtcgaggtgagccccacgttctgcttcactctccccatctcccccccctccccacccccaattttgtatttatttattttttaattattttgtgcagcgatgggggcggggggggggggggggcgcgcgccaggcggggcggggcggggcgaggggcggggcggggcgaggcggagaggtgcggcggcagccaatcagagcggcgcgctccgaaagtttccttttatggcgaggcggcggcggcggcggccctataaaaagcgaagcgcgcggcgggcgggagtcgctgcgacgctgccttcgccccgtgccccgctccgccgccgcctcgcgccgcccgccccggctctgactgaccgcgttactcccacaggtgagcgggcgggacggcccttctcctccgggctgtaattagctgagcaagaggtaagggtttaagggatggttggttggtggggtattaatgtttaattacctggagcacctgcctgaaatcactttttttcaggt

SEQ ID NO: 2 - DNA, 706 bp, synthetic construct
  source 1..706: mol_type = other DNA
cgttacataacttacggtaaatggcccgcctggctgaccgcccaacgacccccgcccattgacgtcaataatgacgtatgttcccatagtaacgccaatagggactttccattgacgtcaatgggtggagtatttacggtaaactgcccacttggcagtacatcaagtgtatcatatgccaagtacgccccctattgacgtcaatgacggtaaatggcccgcctggcattatgcccagtacatgaccttatgggactttcctacttggcagtacatctacgtattagtcatcgctattaccatggctgcagagggccctgcgtatgagtgcaagtgggttttaggaccaggatgaggcggggtgggggtgcctacctgacgaccgaccccgacccactggacaagcacccaacccccattccccaaattgcgcatcccctatcagagagggggaggggaaacaggatgcggcgaggcgcgtgcgcactgccagcttcagcaccgcggacagtgccttcgcccccgcctggcggcgcgcgccaccgccgcctcagcactgaaggcgcgctgacgtcactcgccggtcccccgcaaactccccttcccggccaccttggtcgcgtccgcgccgccgccggcccagccggaccgcaccacgcgaggcgcgagataggggggcacgggcgcgaccatctgcgctgcggcg

SEQ ID NO: 3 - DNA, 580 bp, synthetic construct
  source 1..580: mol_type = other DNA
gacattgattattgactagttattaatagtaatcaattacggggtcattagttcatagcccatatatggagttccgcgttacataacttacggtaaatggcccgcctggctgaccgcccaacgacccccgcccattgacgtcaataatgacgtatgttcccatagtaacgccaatagggactttccattgacgtcaatgggtggagtatttacggtaaactgcccacttggcagtacatcaagtgtatcatatgccaagtacgccccctattgacgtcaatgacggtaaatggcccgcctggcattatgcccagtacatgaccttatgggactttcctacttggcagtacatctacgtattagtcatcgctattaccatggtgatgcggttttggcagtacatcaatgggcgtggatagcggtttgactcacggggatttccaagtctccaccccattgacgtcaatgggagtttgttttggcaccaaaatcaacgggactttccaaaatgtcgtaacaactccgccccattgacgcaaatgggcggtaggcgtgtacggtgggaggtctatataagcag

SEQ ID NO: 4 - DNA, 897 bp, synthetic construct
  source 1..897: mol_type = other DNA
ccattgacgtcaataatgacgtatgttcccatagtaacgccaatagggactttccattgacgtcaatgggtggagtatttacggtaaactgcccacttggcagtacatcaagtgtatcatatgccaagtacgccccctattgacgtcaatgacggtaaatggcccgcctggcattatgcccagtacatgaccttatgggactttcctacttggcagtacatctacgtattagtcatcgctattaccatggtcgaggtgagccccacgttctgcttcactctccccatctcccccccctccccacccccaattttgtatttatttattttttaattattttgtgcagcgatgggggcggggggggggggggggcgcgcgccaggcggggcggggcggggcgaggggcggggcggggcgaggcggagaggtgcggcggcagccaatcagagcggcgcgctccgaaagtttccttttatggcgaggcggcggcggcggcggccctataaaaagcgaagcgcgcggcgggcgggagtcgctgcgcgctgccttcgccccgtgccccgctccgccgccgcctcgcgccgcccgccccggctctgactgaccgcgttactcccacaggtgagcgggcgggacggcccttctcctccgggctgtaattagcgcttggtttaatgacggcttgtttcttttctgtggctgcgtgaaagccttgaggggctccgggagggccctttgtgcggggggagcggctcggggctgtccgcggggggacggctgccttcgggggggacggggcagggcggggttcggcttctggcgtgtgaccggcggctctagagcctctgctaaccatgttcatgccttcttctttttcctacagctcctgggcaacgt

SEQ ID NO: 5 - DNA, 1601 bp, synthetic construct
  source 1..1601: mol_type = other DNA
gttacataacttacggtaaatggcccgcctggctgaccgcccaacgacccccgcccattgacgtcaataatgacgtatgttcccatagtaacgccaatagggactttccattgacgtcaatgggtggagtatttacggtaaactgcccacttggcagtacatcaagtgtatcatatgccaagtacgccccctattgacgtcaatgacggtaaatggcccgcctggcattatgcccagtacatgaccttatgggactttcctacttggcagtacatctacgtattagtcatcgctattaccatggtcgaggtgagccccacgttctgcttcactctccccatctcccccccctccccacccccaattttgtatttatttattttttaattattttgtgcagcgatgggggcggggggggggggggggcgcgcgccaggcggggcggggcggggcgaggggcggggcggggcgaggcggagaggtgcggcggcagccaatcagagcggcgcgctccgaaagtttccttttatggcgaggcggcggcggcggcggccctataaaaagcgaagcgcgcggcgggcggggagtcgctgcgacgctgccttcgccccgtgccccgctccgccgccgcctcgcgccgcccgccccggctctgactgaccgcgttactcccacaggtgagcgggcgggacggcccttctcctccgggctgtaattagcgcttggtttaatgacggcttgtttcttttctgtggctgcgtgaaagccttgaggggctccgggagggccctttgtgcggggggagcggctcggggggtgcgtgcgtgtgtgtgtgcgtggggagcgccgcgtgcggctccgcgctgcccggcggctgtgagcgctgcgggcgcggcgcggggctttgtgcgctccgcagtgtgcgcgaggggagcgcggccgggggcggtgccccgcggtgcggggggggctgcgaggggaacaaaggctgcgtgcggggtgtgtgcgtgggggggtgagcagggggtgtgggcgcgtcggtcgggctgcaaccccccctgcacccccctccccgagttgctgagcacggcccggcttcgggtgcggggctccgtacggggcgtggcgcggggctcgccgtgccgggcggggggtggcggcaggtgggggtgccgggcggggcggggccgcctcgggccggggagggctcgggggaggggcgcggcggcccccggagcgccggcggctgtcgaggcgcggcgagccgcagccattgccttttatggtaatcgtgcgagagggcgcagggacttcctttgtcccaaatctgtgcggagccgaaatctgggaggcgccgccgcaccccctctagcgggcgcggggcgaagcggtgcggcgccggcaggaaggaaatgggcggggagggccttcgtgcgtcgccgcgccgccgtccccttctccctctccagcctcggggctgtccgcggggggacggctgccttcgggggggacggggcagggcggggttcggcttctggcgtgtgaccggcggctctagagcctctgctaaccatgttcatgccttcttctttttcctacag

SEQ ID NO: 6 - DNA, 1052 bp, synthetic construct
  source 1..1052: mol_type = other DNA
gttacataacttacggtaaatggcccgcctggctgaccgcccaacgacccccgcccattgacgtcaataatgacgtatgttcccatagtaacgccaatagggactttccattgacgtcaatgggtggagtatttacggtaaactgcccacttggcagtacatcaagtgtatcatatgccaagtacgccccctattgacgtcaatgacggtaaatggcccgcctggcattatgcccagtacatgaccttatgggactttcctacttggcagtacatctacgtattagtcatcgctattaccatggtcgaggtgagccccacgttctgcttcactctccccatctcccccccctccccacccccaattttgtatttatttattttttaattattttgtgcagcgatgggggcggggggggggggggggcgcgcgccaggcggggcggggcggggcgaggggcggggcggggcgaggcggagaggtgcggcggcagccaatcagagcggcgcgctccgaaagtttccttttatggcgaggcggcggcggcggcggccctataaaaagcgaagcgcgcggcgggcgggagtcgctgcgcgctgccttcgccccgtgccccgctccgccgccgcctcgcgccgcccgccccggctctgactgaccgcgttactaaaacaggtaagtccggcctccgcgccgggttttggcgcctcccgcgggcgcccccctcctcacggcgagcgctgccacgtcagacgaagggcgcagcgagcgtcctgatccttccgcccggacgctcaggacagcggcccgctgctcataagactcggccttagaaccccagtatcagcagaaggacattttaggacgggacttgggtgactctagggcactggttttctttccagagagcggaacaggcgaggaaaagtagtcccttctcggcgattctgcggagggatctccgtggggcggtgaacgccgatgatgcctctactaaccatgttcatgttttctttttttttctacaggtcctgggtgacgaacaggctagc

SEQ ID NO: 7 - protein, 480 aa, Homo sapiens
MNASEFRRRGKEMVDYMANYMEGIEGRQVYPDVEPGYLRPLIPAAAPQEPDTFEDIINDVEKIIMPGVTHWHSPYFFAYFPTASSYPAMLADMLCGAIGCIGFSWAASPACTELETVMMDWLGKMLELPKAFLNEKAGEGGGVIQGSASEATLVALLAARTKVIHRLQAASPELTQAAIMEKLVAYSSDQAHSSVERAGLIGGVKLKAIPSDGNFAMRASALQEALERDKAAGLIPFFMVATLGTTTCCSFDNLLEVGPICNKEDIWLHVDAAYAGSAFICPEFRHLLNGVEFADSFNFNPHKWLLVNFDCSAMWVKKRTDLTGAFRLDPTYLKHSHQDSGLITDYRHWQIPLGRRFRSLKMWFVFRMYGVKGLQAYIRKHVQLSHEFESLVRQDPRFEICVEVILGLVCFRLKGSNKVNEALLQRINSAKKIHLVPCHLRDKFVLRFAICSRTVESAHVQRAWEHIKELAADVLRAERE

SEQ ID NO: 8 - DNA, 1440 bp, synthetic construct
  source 1..1440: mol_type = other DNA
atgaacgcaagtgaattccgaaggagagggaaggagatggtggattacatggccaactacatggaaggcattgagggacgccaggtctaccctgacgtggagcccgggtacctgcggccgctgatccctgccgctgcccctcaggagccagacacgtttgaggacatcatcaacgacgttgagaagataatcatgcctggggtgacgcactggcacagcccctacttcttcgcctacttccccactgccagctcgtacccggccatgcttgcggacatgctgtgcggggccattggctgcatcggcttctcctgggcggcaagcccagcatgcacagagctggagactgtgatgatggactggctcgggaagatgctggaactaccaaaggcatttttgaatgagaaagctggagaagggggaggagtgatccagggaagtgccagtgaagccaccctggtggccctgctggccgctcggaccaaagtgatccatcggctgcaggcagcgtccccagagctcacacaggccgctatcatggagaagctggtggcttactcatccgatcaggcacactcctcagtggaaagagctgggttaattggtggagtgaaattaaaagccatcccctcagatggcaacttcgccatgcgtgcgtctgccctgcaggaagccctggagagagacaaagcggctggcctgattcctttctttatggttgccaccctggggaccacaacatgctgctcctttgacaatctcttagaagtcggtcctatctgcaacaaggaagacatatggctgcacgttgatgcagcctacgcaggcagtgcattcatctgccctgagttccggcaccttctgaatggagtggagtttgcagattcattcaactttaatccccacaaatggctattggtgaattttgactgttctgccatgtgggtgaaaaagagaacagacttaacgggagcctttagactggaccccacttacctgaagcacagccatcaggattcagggcttatcactgactaccggcattggcagataccactgggcagaagatttcgctctttgaaaatgtggtttgtatttaggatgtatggagtcaaaggactgcaggcttatatccgcaagcatgtccagctgtcccatgagtttgagtcactggtgcgccaggatccccgctttgaaatctgtgtggaagtcattctggggcttgtctgctttcggctaaagggttccaacaaagtgaatgaagctcttctgcaaagaataaacagtgccaaaaaaatccacttggttccatgtcacctcagggacaagtttgtcctgcgctttgccatctgttctcgcacggtggaatctgcccatgtgcagcgggcctgggaacacatcaaagagctggcggccgacgtgctgcgagcagagagggag

SEQ ID NO: 9 - protein, 250 aa, Homo sapiens
MEKGPVRAPAEKPRGARCSNGFPERDPPRPGPSRPAEKPPRPEAKSAQPADGWKGERPRSEEDNELNLPNLAAAYSSILSSLGENPQRQGLLKTPWRAASAMQFFTKGYQETISDVLNDAIFDEDHDEMVIVKDIDMFSMCEHHLVPFVGKVHIGYLPNKQVLGLSKLARIVEIYSRRLQVQERLTKQIAVAITEALRPAGVGVVVEATHMCMVMRGVQKMNSKTVTSTMLGVFREDPKTREEFLTLIRS

SEQ ID NO: 10 - DNA, 750 bp, synthetic construct
  source 1..750: mol_type = other DNA
atggagaagggccctgtgcgggcaccggcggagaagccgcggggcgccaggtgcagcaatgggttccccgagcgggatccgccgcggcccgggcccagcaggccggcggagaagcccccgcggcccgaggccaagagcgcgcagcccgcggacggctggaagggcgagcggccccgcagcgaggaggataacgagctgaacctccctaacctggcagccgcctactcgtccatcctgagctcgctgggcgagaacccccagcggcaagggctgctcaagacgccctggagggcggcctcggccatgcagttcttcaccaagggctaccaggagaccatctcagatgtcctaaacgatgctatatttgatgaagatcatgatgagatggtgattgtgaaggacatagacatgttttccatgtgtgagcatcacttggttccatttgttggaaaggtccatattggttatcttcctaacaagcaagtccttggcctcagcaaacttgcgaggattgtagaaatctatagtagaagactacaagttcaggagcgccttacaaaacaaattgctgtagcaatcacggaagccttgcggcctgctggagtcggggtagtggttgaagcaacacacatgtgtatggtaatgcgaggtgtacagaaaatgaacagcaaaactgtgaccagcacaatgttgggtgtgttccgggaggatccaaagactcgggaagagttcctgactctcattaggagc

SEQ ID NO: 11 - protein, 338 aa, Homo sapiens
MVKVPWFPRKVSELDKCHHLVTKFDPDLDLDHPGFSDQVYRQRRKLIAEIAFQYRHGDPIPRVEYTAEEIATWKEVYTTLKGLYATHACGEHLEAFALLERFSGYREDNIPQLEDVSRFLKERTGFQLRPVAGLLSARDFLASLAFRVFQCTQYIRHASSPMHSPEPDCCHELLGHVPMLADRTFAQFSQDIGLASLGASDEEIEKLSTLYWFTVEFGLCKQNGEVKAYGAGLLSSYGELLHCLSEEPEIRAFDPEAAAVQPYQDQTYQSVYFVSESFSDAKDKLRSYASRIQRPFSVKFDPYTLAIDVLDSPQAVRRSLEGVQDELDTLAHALSAIG

SEQ ID NO: 12 - DNA, 1014 bp, synthetic construct
  source 1..1014: mol_type = other DNA
atggtgaaggtcccctggttcccaagaaaagtgtcagagctggacaagtgtcatcacctggtcaccaagttcgaccctgacctggacttggaccacccgggcttctcggaccaggtgtaccgccagcgcaggaagctgattgctgagatcgccttccagtacaggcacggcgacccgattccccgtgtggagtacaccgccgaggagattgccacctggaaggaggtctacaccacgctgaagggcctctacgccacgcacgcctgcggggagcacctggaggcctttgctttgctggagcgcttcagcggctaccgggaagacaatatcccccagctggaggacgtctcccgcttcctgaaggagcgcacgggcttccagctgcggcctgtggccggcctgctgtccgcccgggacttcctggccagcctggccttccgcgtgttccagtgcacccagtatatccgccacgcgtcctcgcccatgcactcccctgagccggactgctgccacgagctgctggggcacgtgcccatgctggccgaccgcaccttcgcgcagttctcgcaggacattggcctggcgtccctgggggcctcggatgaggaaattgagaagctgtccacgctgtactggttcacggtggagttcgggctgtgtaagcagaacggggaggtgaaggcctatggtgccgggctgctgtcctcctacggggagctcctgcactgcctgtctgaggagcctgagattcgggccttcgaccctgaggctgcggccgtgcagccctaccaagaccagacgtaccagtcagtctacttcgtgtctgagagcttcagtgacgccaaggacaagctcaggagctatgcctcacgcatccagcgccccttctccgtgaagttcgacccgtacacgctggccatcgacgtgctggacagcccccaggccgtgcggcgctccctggagggtgtccaggatgagctggacacccttgcccatgcgctgagtgccattgga

SEQ ID NO: 13 - protein, 22 aa, synthetic construct
GSGATNFSLLKQAGDVEENPGP

SEQ ID NO: 14 - DNA, 66 bp, synthetic construct
  source 1..66: mol_type = other DNA
ggaagcggagctactaacttcagcctgctgaagcaggctggcgacgtggaggagaaccctggacct

SEQ ID NO: 15 - protein, 25 aa, synthetic construct
GSGVKQTLNFDLLKLAGDVESNPGP

SEQ ID NO: 16 - DNA, 75 bp, synthetic construct
  source 1..75: mol_type = other DNA
ggaagcggagtgaaacagactttgaattttgaccttctcaagttggcgggagacgtggagtccaaccctggacct

SEQ ID NO: 17 - protein, 15 aa, synthetic construct
GGGGSGGGGSGGGGS

SEQ ID NO: 18 - DNA, 45 bp, synthetic construct
  source 1..45: mol_type = other DNA
ggaggcggcggctctggtggaggcggcagcggcggcggcggttct

SEQ ID NO: 19 - DNA, 3339 bp, synthetic construct
  source 1..3339: mol_type = other DNA
atgaacgcaagtgaattccgaaggagagggaaggagatggtggattacatggccaactacatggaaggcattgagggacgccaggtctaccctgacgtggagcccgggtacctgcggccgctgatccctgccgctgcccctcaggagccagacacgtttgaggacatcatcaacgacgttgagaagataatcatgcctggggtgacgcactggcacagcccctacttcttcgcctacttccccactgccagctcgtacccggccatgcttgcggacatgctgtgcggggccattggctgcatcggcttctcctgggcggcaagcccagcatgcacagagctggagactgtgatgatggactggctcgggaagatgctggaactaccaaaggcatttttgaatgagaaagctggagaagggggaggagtgatccagggaagtgccagtgaagccaccctggtggccctgctggccgctcggaccaaagtgatccatcggctgcaggcagcgtccccagagctcacacaggccgctatcatggagaagctggtggcttactcatccgatcaggcacactcctcagtggaaagagctgggttaattggtggagtgaaattaaaagccatcccctcagatggcaacttcgccatgcgtgcgtctgccctgcaggaagccctggagagagacaaagcggctggcctgattcctttctttatggttgccaccctggggaccacaacatgctgctcctttgacaatctcttagaagtcggtcctatctgcaacaaggaagacatatggctgcacgttgatgcagcctacgcaggcagtgcattcatctgccctgagttccggcaccttctgaatggagtggagtttgcagattcattcaactttaatccccacaaatggctattggtgaattttgactgttctgccatgtgggtgaaaaagagaacagacttaacgggagcctttagactggaccccacttacctgaagcacagccatcaggattcagggcttatcactgactaccggcattggcagataccactgggcagaagatttcgctctttgaaaatgtggtttgtatttaggatgtatggagtcaaaggactgcaggcttatatccgcaagcatgtccagctgtcccatgagtttgagtcactggtgcgccaggatccccgctttgaaatctgtgtggaagtcattctggggcttgtctgctttcggctaaagggttccaacaaagtgaatgaagctcttctgcaaagaataaacagtgccaaaaaaatccacttggttccatgtcacctcagggacaagtttgtcctgcgctttgccatctgttctcgcacggtggaatctgcccatgtgcagcgggcctgggaacacatcaaagagctggcggccgacgtgctgcgagcagagagggagggaagcggagctactaacttcagcctgctgaagcaggctggcgacgtggaggagaaccctggacctatggagaagggccctgtgcgggcaccggcggagaagccgcggggcgccaggtgcagcaatgggttccccgagcgggatccgccgcggcccgggcccagcaggccggcggagaagcccccgcggcccgaggccaagagcgcgcagcccgcggacggctggaagggcgagcggccccgcagcgaggaggataacgagctgaacctccctaacctggcagccgcctactcgtccatcctgagctcgctgggcgagaacccccagcggcaagggctgctcaagacgccctggagggcggcctcggccatgcagttcttcaccaagggctaccaggagaccatctcagatgtcctaaacgatgctatatttgatgaagatcatgatgagatggtgattgtgaaggacatagacatgttttccatgtgtgagcatcacttggttccatttgttggaaaggtccatattggttatcttcctaacaagcaagtccttggcctcagcaaacttgcgaggattgtagaaatctatagtagaagactacaagttcaggagcgccttacaaaacaaattgctgtagcaatcacggaagccttgcggcctgctggagtcggggtagtggttgaagcaacacacatgtgtatggtaatgcgaggtgtacagaaaatgaacagcaaaactgtgaccagcacaatgttgggtgtgttccgggaggatccaaagactcgggaagagttcctgactctcattaggagcggaagcggagctactaacttcagcctgctgaagcaggctggcgacgtggaggagaaccctggacctatggtgaaggtaccctggttcccaagaaaagtgtcagagctggacaagtgtcatcacctggtcaccaagttcgaccccgacctggacttggaccaccccggcttctcggaccaggtgtaccgccagcgcaggaagctgatcgctgagatcgccttccagtacaggcacggcgacccgatcccccgtgtggagtacaccgccgaggagatcgccacctggaaggaggtctacaccaccctgaagggcctctacgccacccacgcctgcggggagcacctggaggcctttgctttgctggagcgcttcagcggctaccgggaagacaacatcccccagctggaggacgtctcccgcttcctgaaggagcgcacaggcttccagctgcggcccgtggccggcctgctgtccgcccgggacttcctggccagcctggccttccgcgtgttccagtgcacccagtatatccgccacgcgtcctcgcccatgcactcccctgagccggactgctgccacgagctgctggggcacgtgcccatgctggccgaccgcaccttcgcgcagttcagccaggacatcggcctggcgtccctgggggccagcgatgaggaaatcgagaagctgtccactctgtactggttcacggtggagttcgggctgtgtaagcagaacggggaggtgaaggcctatggtgccgggctgctgtcctcctacggggagctcctgcactgcctgtctgaggagcctgagatccgggccttcgaccctgaggctgcggccgtgcagccctaccaagaccagacgtaccagtcagtctacttcgtgtctgagagcttcagcgacgccaaggacaagctcaggagctatgccagccgcatccagcgccccttctccgtgaagttcgacccgtacaccctggccatcgacgtgctggacagcccccaggccgtgcggcgctccctggagggtgtccaggatgagctggacacccttgcccatgcgctgagcgccatcggctga

SEQ ID NO: 20 - DNA, 3318 bp, synthetic construct
  source 1..3318: mol_type = other DNA
atggtgaaggtcccctggttcccaagaaaagtgtcagagctggacaagtgtcatcacctggtcaccaagttcgaccctgacctggacttggaccacccgggcttctcggaccaggtgtaccgccagcgcaggaagctgattgctgagatcgccttccagtacaggcacggcgacccgattccccgtgtggagtacaccgccgaggagattgccacctggaaggaggtctacaccacgctgaagggcctctacgccacgcacgcctgcggggagcacctggaggcctttgctttgctggagcgcttcagcggctaccgggaagacaatatcccccagctggaggacgtctcccgcttcctgaaggagcgcacgggcttccagctgcggcctgtggccggcctgctgtccgcccgggacttcctggccagcctggccttccgcgtgttccagtgcacccagtatatccgccacgcgtcctcgcccatgcactcccctgagccggactgctgccacgagctgctggggcacgtgcccatgctggccgaccgcaccttcgcgcagttctcgcaggacattggcctggcgtccctgggggcctcggatgaggaaattgagaagctgtccacgctgtactggttcacggtggagttcgggctgtgtaagcagaacggggaggtgaaggcctatggtgccgggctgctgtcctcctacggggagctcctgcactgcctgtctgaggagcctgagattcgggccttcgaccctgaggctgcggccgtgcagccctaccaagaccagacgtaccagtcagtctacttcgtgtctgagagcttcagtgacgccaaggacaagctcaggagctatgcctcacgcatccagcgccccttctccgtgaagttcgacccgtacacgctggccatcgacgtgctggacagcccccaggccgtgcggcgctccctggagggtgtccaggatgagctggacacccttgcccatgcgctgagtgccattggaggaggcggcggctctggtggaggcggcagcggcggcggcggttctatggagaagggccctgtgcgggcaccggcggagaagccgcggggcgccaggtgcagcaatgggttccccgagcgggatccgccgcggcccgggcccagcaggccggcggagaagcccccgcggcccgaggccaagagcgcgcagcccgcggacggctggaagggcgagcggccccgcagcgaggaggataacgagctgaacctccctaacctggcagccgcctactcgtccatcctgagctcgctgggcgagaacccccagcggcaagggctgctcaagacgccctggagggcggcctcggccatgcagttcttcaccaagggctaccaggagaccatctcagatgtcctaaacgatgctatatttgatgaagatcatgatgagatggtgattgtgaaggacatagacatgttttccatgtgtgagcatcacttggttccatttgttggaaaggtccatattggttatcttcctaacaagcaagtccttggcctcagcaaacttgcgaggattgtagaaatctatagtagaagactacaagttcaggagcgccttacaaaacaaattgctgtagcaatcacggaagccttgcggcctgctggagtcggggtagtggttgaagcaacacacatgtgtatggtaatgcgaggtgtacagaaaatgaacagcaaaactgtgaccagcacaatgttgggtgtgttccgggaggatccaaagactcgggaagagttcctgactctcattaggagcggaagcggagctactaacttcagcctgctgaagcaggctggcgacgtggaggagaaccctggacctatgaacgcaagtgaattccgaaggagagggaaggagatggtggattacatggccaactacatggaaggcattgagggacgccaggtctaccctgacgtggagcccgggtacctgcggccgctgatccctgccgctgcccctcaggagccagacacgtttgaggacatcatcaacgacgttgagaagataatcatgcctggggtgacgcactggcacagcccctacttcttcgcctacttccccactgccagctcgtacccggccatgcttgcggacatgctgtgcggggccattggctgcatcggcttctcctgggcggcaagcccagcatgcacagagctggagactgtgatgatggactggctcgggaagatgctggaactaccaaaggcatttttgaatgagaaagctggagaagggggaggagtgatccagggaagtgccagtgaagccaccctggtggccctgctggccgctcggaccaaagtgatccatcggctgcaggcagcgtccccagagctcacacaggccgctatcatggagaagctggtggcttactcatccgatcaggcacactcctcagtggaaagagctgggttaattggtggagtgaaattaaaagccatcccctcagatggcaacttcgccatgcgtgcgtctgccctgcaggaagccctggagagagacaaagcggctggcctgattcctttctttatggttgccaccctggggaccacaacatgctgctcctttgacaatctcttagaagtcggtcctatctgcaacaaggaagacatatggctgcacgttgatgcagcctacgcaggcagtgcattcatctgccctgagttccggcaccttctgaatggagtggagtttgcagattcattcaactttaatccccacaaatggctattggtgaattttgactgttctgccatgtgggtgaaaaagagaacagacttaacgggagcctttagactggaccccacttacctgaagcacagccatcaggattcagggcttatcactgactaccggcattggcagataccactgggcagaagatttcgctctttgaaaatgtggtttgtatttaggatgtatggagtcaaaggactgcaggcttatatccgcaagcatgtccagctgtcccatgagtttgagtcactggtgcgccaggatccccgctttgaaatctgtgtggaagtcattctggggcttgtctgctttcggctaaagggttccaacaaagtgaatgaagctcttctgcaaagaataaacagtgccaaaaaaatccacttggttccatgtcacctcagggacaagtttgtcctgcgctttgccatctgttctcgcacggtggaatctgcccatgtgcagcgggcctgggaacacatcaaagagctggcggccgacgtgctgcgagcagagagggagtga

SEQ ID NO: 21 - DNA, 3348 bp, synthetic construct
  source 1..3348: mol_type = other DNA
atggtgaaggtcccctggttcccaagaaaagtgtcagagctggacaagtgtcatcacctggtcaccaagttcgaccctgacctggacttggaccacccgggcttctcggaccaggtgtaccgccagcgcaggaagctgattgctgagatcgccttccagtacaggcacggcgacccgattccccgtgtggagtacaccgccgaggagattgccacctggaaggaggtctacaccacgctgaagggcctctacgccacgcacgcctgcggggagcacctggaggcctttgctttgctggagcgcttcagcggctaccgggaagacaatatcccccagctggaggacgtctcccgcttcctgaaggagcgcacgggcttccagctgcggcctgtggccggcctgctgtccgcccgggacttcctggccagcctggccttccgcgtgttccagtgcacccagtatatccgccacgcgtcctcgcccatgcactcccctgagccggactgctgccacgagctgctggggcacgtgcccatgctggccgaccgcaccttcgcgcagttctcgcaggacattggcctggcgtccctgggggcctcggatgaggaaattgagaagctgtccacgctgtactggttcacggtggagttcgggctgtgtaagcagaacggggaggtgaaggcctatggtgccgggctgctgtcctcctacggggagctcctgcactgcctgtctgaggagcctgagattcgggccttcgaccctgaggctgcggccgtgcagccctaccaagaccagacgtaccagtcagtctacttcgtgtctgagagcttcagtgacgccaaggacaagctcaggagctatgcctcacgcatccagcgccccttctccgtgaagttcgacccgtacacgctggccatcgacgtgctggacagcccccaggccgtgcggcgctccctggagggtgtccaggatgagctggacacccttgcccatgcgctgagtgccattggaggaagcggagtgaaacagactttgaattttgaccttctcaagttggcgggagacgtggagtccaaccctggacctatggagaagggccctgtgcgggcaccggcggagaagccgcggggcgccaggtgcagcaatgggttccccgagcgggatccgccgcggcccgggcccagcaggccggcggagaagcccccgcggcccgaggccaagagcgcgcagcccgcggacggctggaagggcgagcggccccgcagcgaggaggataacgagctgaacctccctaacctggcagccgcctactcgtccatcctgagctcgctgggcgagaacccccagcggcaagggctgctcaagacgccctggagggcggcctcggccatgcagttcttcaccaagggctaccaggagaccatctcagatgtcctaaacgatgctatatttgatgaagatcatgatgagatggtgattgtgaaggacatagacatgttttccatgtgtgagcatcacttggttccatttgttggaaaggtccatattggttatcttcctaacaagcaagtccttggcctcagcaaacttgcgaggattgtagaaatctatagtagaagactacaagttcaggagcgccttacaaaacaaattgctgtagcaatcacggaagccttgcggcctgctggagtcggggtagtggttgaagcaacacacatgtgtatggtaatgcgaggtgtacagaaaatgaacagcaaaactgtgaccagcacaatgttgggtgtgttccgggaggatccaaagactcgggaagagttcctgactctcattaggagcggaagcggagctactaacttcagcctgctgaagcaggctggcgacgtggaggagaaccctggacctatgaacgcaagtgaattccgaaggagagggaaggagatggtggattacatggccaactacatggaaggcattgagggacgccaggtctaccctgacgtggagcccgggtacctgcggccgctgatccctgccgctgcccctcaggagccagacacgtttgaggacatcatcaacgacgttgagaagataatcatgcctggggtgacgcactggcacagcccctacttcttcgcctacttccccactgccagctcgtacccggccatgcttgcggacatgctgtgcggggccattggctgcatcggcttctcctgggcggcaagcccagcatgcacagagctggagactgtgatgatggactggctcgggaagatgctggaactaccaaaggcatttttgaatgagaaagctggagaagggggaggagtgatccagggaagtgccagtgaagccaccctggtggccctgctggccgctcggaccaaagtgatccatcggctgcaggcagcgtccccagagctcacacaggccgctatcatggagaagctggtggcttactcatccgatcaggcacactcctcagtggaaagagctgggttaattggtggagtgaaattaaaagccatcccctcagatggcaacttcgccatgcgtgcgtctgccctgcaggaagccctggagagagacaaagcggctggcctgattcctttctttatggttgccaccctggggaccacaacatgctgctcctttgacaatctcttagaagtcggtcctatctgcaacaaggaagacatatggctgcacgttgatgcagcctacgcaggcagtgcattcatctgccctgagttccggcaccttctgaatggagtggagtttgcagattcattcaactttaatccccacaaatggctattggtgaattttgactgttctgccatgtgggtgaaaaagagaacagacttaacgggagcctttagactggaccccacttacctgaagcacagccatcaggattcagggcttatcactgactaccggcattggcagataccactgggcagaagatttcgctctttgaaaatgtggtttgtatttaggatgtatggagtcaaaggactgcaggcttatatccgcaagcatgtccagctgtcccatgagtttgagtcactggtgcgccaggatccccgctttgaaatctgtgtggaagtcattctggggcttgtctgctttcggctaaagggttccaacaaagtgaatgaagctcttctgcaaagaataaacagtgccaaaaaaatccacttggttccatgtcacctcagggacaagtttgtcctgcgctttgccatctgttctcgcacggtggaatctgcccatgtgcagcgggcctgggaacacatcaaagagctggcggccgacgtgctgcgagcagagagggagtga

SEQ ID NO: 22 - DNA, 3763 bp, synthetic construct
  source 1..3763: mol_type = other DNA
accggtcgccaccgtcgacgtttatttgtgaaatttgtgatgctattgctttatttgtaaccattataagctgcaataaacaagttaacaacaacaattgcattcattttatgtttcaggttcagggggagatgtgggaggttttttaaagtttaaacaggaacccctagtgatggagttggccactccctctctgcgcgctcgctcgctcactgaggccgggcgaccaaaggtcgcccgacgcccgggctttgcccgggcggcctcagtgagcgagcgagcgcgcagctgcctgcaggacatgtgagcaaaaggccagcaaaaggccaggaaccgtaagcttaaaaaggccgcgttgctggcgtttttccataggctccgcccccctgacgagcatcacaaaaatcgacgctcaagtcagaggtggcgaaacccgacaggactataaagataccaggcgtttccccctggaagctccctcgtgcgctctcctgttccgaccctgccgcttaccggatacctgtccgcctttctcccttcgggaagcgtggcgctttctcatagctcacgctgtaggtatctcagttcggtgtaggtcgttcgctccaagctgggctgtgtgcacgaaccccccgttcagcccgaccgctgcgccttatccggtaactatcgtcttgagtccaacccggtaagacacgacttatcgccactggcagcagccactggtaacaggattagcagagcgaggtatgtaggcggtgctacagagttcttgaagtggtggcctaactacggctacactagaagaacagtatttggtatctgcgctctgctgaagccagttaccttcggaaaaagagttggtagctcttgatccggcaaacaaaccaccgctggtagcggtggtttttttgtttgcaagcagcagattacgcgcagaaaaaaaggatctcaagaagatcctttgatcttttctacggggtctgacgctcagtggaacgaaaactcacgttaagggattttggtcatgagattatcaaaaaggatcttcacctagatccttttaaattaaaaatgaagttttaaatcaagcccaatctgaataatgttacaaccaattaaccaattctgattagaaaaactcatcgagcatcaaatgaaactgcaatttattcatatcaggattatcaataccatatttttgaaaaagccgtttctgtaatgaaggagaaaactcaccgaggcagttccataggatggcaagatcctggtatcggtctgcgattccgactcgtccaacatcaatacaacctattaatttcccctcgtcaaaaataaggttatcaagtgagaaatcaccatgagtgacgactgaatccggtgagaatggcaaaagtttatgcatttctttccagacttgttcaacaggccagccattacgctcgtcatcaaaatcactcgcatcaaccaaaccgttattcattcgtgattgcgcctgagcgagacgaaatacgcgatcgctgttaaaaggacaattacaaacaggaatcgaatgcaaccggcgcaggaacactgccagcgcatcaacaatattttcacctgaatcaggatattcttctaatacctggaatgctgtttttccggggatcgcagtggtgagtaaccatgcatcatcaggagtacggataaaatgcttgatggtcggaagaggcataaattccgtcagccagtttagtctgaccatctcatctgtaacatcattggcaacgctacctttgccatgtttcagaaacaactctggcgcatcgggcttcccatacaagcgatagattgtcgcacctgattgcccgacattatcgcgagcccatttatacccatataaatcagcatccatgttggaatttaatcgcggcctcgacgtttcccgttgaatatggctcataacaccccttgtattactgtttatgtaagcagacagttttattgttcatgatgatatatttttatcttgtgcaatgtaacatcagagattttgagacacgggccagagctgcatcgcgcgtttcggtgatgacggtgaaaacctctgacacatgcagctcccggagacggtcacagcttgtctgtaagcggatgccgggagcagacaagcccgtcagggcgcgtcagcgggtgttggcgggtgtcggggctggcttaactatgcggcatcagagcagattgtactgagagtgcaccataaaattgtaaacgttaatattttgttaaaattcgcgttaaatttttgttaaatcagctcattttttaaccaataggccgaaatcggcaaaatcccttataaatcaaaagaatagcccgagatagggttgagtgttgttccagtttggaacaagagtccactattaaagaacgtggactccaacgtcaaagggcgaaaaaccgtctatcagggcgatggcccactacgtgaaccatcacccaaatcaagttttttggggtcgaggtgccgtaaagcactaaatcggaaccctaaagggagcccccgatttagagcttgacggggaaagccggcgaacgtggcgagaaaggaagggaagaaagcgaaaggagcgggcgctagggcgctggcaagtgtagcggtcacgctgcgcgtaaccaccacacccgccgcgcttaatgcgggtaccccgctacagggcgcgtactatggttgctttgacgtatgcggtgtgaaataccgcacagatgcgtaaggagaaaataccgcatcaggcgcccctgcaggcagctgcgcgctcgctcgctcactgaggccgcccgggcaaagcccgggcgtcgggcgacctttggtcgcccggcctcagtgagcgagcgagcgcgcagagagggagtggccaactccatcactaggggttcctacgcgtcgttacataacttacggtaaatggcccgcctggctgaccgcccaacgacccccgcccattgacgtcaataatgacgtatgttcccatagtaacgccaatagggactttccattgacgtcaatgggtggagtatttacggtaaactgcccacttggcagtacatcaagtgtatcatatgccaagtacgccccctattgacgtcaatgacggtaaatggcccgcctggcattatgcccagtacatgaccttatgggactttcctacttggcagtacatctacgtattagtcatcgctattaccatggtcgaggtgagccccacgttctgcttcactctccccatctcccccccctccccacccccaattttgtatttatttattttttaattattttgtgcagcgatgggggcgggggggggggggggcgcgcgccaggcggggcggggcggggcgaggggcggggcggggcgaggcggagaggtgcggcggcagccaatcagagcggcgcgctccgaaagtttccttttatggcgaggcggcggcggcggcggccctataaaaagcgaagcgcgcggcgggcgggagtcgctgcgcgctgccttcgccccgtgccccgctccgccgccgcctcgcgccgcccgccccggctctgactgaccgcgttactcccacaggtgagcgggcgggacggcccttctcctccgggctgtaattagctgagcaagaggtaagggtttaagggatggttggttggtggggtattaatgtttaattacctggagcacctgcctgaaatcactttttttcaggtacacccaagctgtctagagccgccacc

SEQ ID NO: 23 - DNA, 4483 bp, synthetic construct
  source 1..4483: mol_type = other DNA
accggtcgccaccatggtgagcaagggcgaggagctgttcaccggggtggtgcccatcctggtcgagctggacggcgacgtaaacggccacaagttcagcgtgtccggcgagggcgagggcgatgccacctacggcaagctgaccctgaagttcatctgcaccaccggcaagctgcccgtgccctggcccaccctcgtgaccaccctgacctacggcgtgcagtgcttcagccgctaccccgaccacatgaagcagcacgacttcttcaagtccgccatgcccgaaggctacgtccaggagcgcaccatcttcttcaaggacgacggcaactacaagacccgcgccgaggtgaagttcgagggcgacaccctggtgaaccgcatcgagctgaagggcatcgacttcaaggaggacggcaacatcctggggcacaagctggagtacaactacaacagccacaacgtctatatcatggccgacaagcagaagaacggcatcaaggtgaacttcaagatccgccacaacatcgaggacggcagcgtgcagctcgccgaccactaccagcagaacacccccatcggcgacggccccgtgctgctgcccgacaaccactacctgagcacccagtccgccctgagcaaagaccccaacgagaagcgcgatcacatggtcctgctggagttcgtgaccgccgccgggatcactctcggcatggacgagctgtacaagtaggtcgacgtttatttgtgaaatttgtgatgctattgctttatttgtaaccattataagctgcaataaacaagttaacaacaacaattgcattcattttatgtttcaggttcagggggagatgtgggaggttttttaaagtttaaacaggaacccctagtgatggagttggccactccctctctgcgcgctcgctcgctcactgaggccgggcgaccaaaggtcgcccgacgcccgggctttgcccgggcggcctcagtgagcgagcgagcgcgcagctgcctgcaggacatgtgagcaaaaggccagcaaaaggccaggaaccgtaagcttaaaaaggccgcgttgctggcgtttttccataggctccgcccccctgacgagcatcacaaaaatcgacgctcaagtcagaggtggcgaaacccgacaggactataaagataccaggcgtttccccctggaagctccctcgtgcgctctcctgttccgaccctgccgcttaccggatacctgtccgcctttctcccttcgggaagcgtggcgctttctcatagctcacgctgtaggtatctcagttcggtgtaggtcgttcgctccaagctgggctgtgtgcacgaaccccccgttcagcccgaccgctgcgccttatccggtaactatcgtcttgagtccaacccggtaagacacgacttatcgccactggcagcagccactggtaacaggattagcagagcgaggtatgtaggcggtgctacagagttcttgaagtggtggcctaactacggctacactagaagaacagtatttggtatctgcgctctgctgaagccagttaccttcggaaaaagagttggtagctcttgatccggcaaacaaaccaccgctggtagcggtggtttttttgtttgcaagcagcagattacgcgcagaaaaaaaggatctcaagaagatcctttgatcttttctacggggtctgacgctcagtggaacgaaaactcacgttaagggattttggtcatgagattatcaaaaaggatcttcacctagatccttttaaattaaaaatgaagttttaaatcaagcccaatctgaataatgttacaaccaattaaccaattctgattagaaaaactcatcgagcatcaaatgaaactgcaatttattcatatcaggattatcaataccatatttttgaaaaagccgtttctgtaatgaaggagaaaactcaccgaggcagttccataggatggcaagatcctggtatcggtctgcgattccgactcgtccaacatcaatacaacctattaatttcccctcgtcaaaaataaggttatcaagtgagaaatcaccatgagtgacgactgaatccggtgagaatggcaaaagtttatgcatttctttccagacttgttcaacaggccagccattacgctcgtcatcaaaatcactcgcatcaaccaaaccgttattcattcgtgattgcgcctgagcgagacgaaatacgcgatcgctgttaaaaggacaattacaaacaggaatcgaatgcaaccggcgcaggaacactgccagcgcatcaacaatattttcacctgaatcaggatattcttctaatacctggaatgctgtttttccggggatcgcagtggtgagtaaccatgcatcatcaggagtacggataaaatgcttgatggtcggaagaggcataaattccgtcagccagtttagtctgaccatctcatctgtaacatcattggcaacgctacctttgccatgtttcagaaacaactctggcgcatcgggcttcccatacaagcgatagattgtcgcacctgattgcccgacattatcgcgagcccatttatacccatataaatcagcatccatgttggaatttaatcgcggcctcgacgtttcccgttgaatatggctcataacaccccttgtattactgtttatgtaagcagacagttttattgttcatgatgatatatttttatcttgtgcaatgtaacatcagagattttgagacacgggccagagctgcatcgcgcgtttcggtgatgacggtgaaaacctctgacacatgcagctcccggagacggtcacagcttgtctgtaagcggatgccgggagcagacaagcccgtcagggcgcgtcagcgggtgttggcgggtgtcggggctggcttaactatgcggcatcagagcagattgtactgagagtgcaccataaaattgtaaacgttaatattttgttaaaattcgcgttaaatttttgttaaatcagctcattttttaaccaataggccgaaatcggcaaaatcccttataaatcaaaagaatagcccgagatagggttgagtgttgttccagtttggaacaagagtccactattaaagaacgtggactccaacgtcaaagggcgaaaaaccgtctatcagggcgatggcccactacgtgaaccatcacccaaatcaagttttttggggtcgaggtgccgtaaagcactaaatcggaaccctaaagggagcccccgatttagagcttgacggggaaagccggcgaacgtggcgagaaaggaagggaagaaagcgaaaggagcgggcgctagggcgctggcaagtgtagcggtcacgctgcgcgtaaccaccacacccgccgcgcttaatgcgggtaccccgctacagggcgcgtactatggttgctttgacgtatgcggtgtgaaataccgcacagatgcgtaaggagaaaataccgcatcaggcgcccctgcaggcagctgcgcgctcgctcgctcactgaggccgcccgggcaaagcccgggcgtcgggcgacctttggtcgcccggcctcagtgagcgagcgagcgcgcagagagggagtggccaactccatcactaggggttcctacgcgtcgttacataacttacggtaaatggcccgcctggctgaccgcccaacgacccccgcccattgacgtcaataatgacgtatgttcccatagtaacgccaatagggactttccattgacgtcaatgggtggagtatttacggtaaactgcccacttggcagtacatcaagtgtatcatatgccaagtacgccccctattgacgtcaatgacggtaaatggcccgcctggcattatgcccagtacatgaccttatgggactttcctacttggcagtacatctacgtattagtcatcgctattaccatggtcgaggtgagccccacgttctgcttcactctccccatctcccccccctccccacccccaattttgtatttatttattttttaattattttgtgcagcgatgggggcgggggggggggggggcgcgcgccaggcggggcggggcggggcgaggggcggggcggggcgaggcggagaggtgcggcggcagccaatcagagcggcgcgctccgaaagtttccttttatggcgaggcggcggcggcggcggccctataaaaagcgaagcgcgcggcgggcgggagtcgctgcgcgctgccttcgccccgtgccccgctccgccgccgcctcgcgccgcccgccccggctctgactgaccgcgttactcccacaggtgagcgggcgggacggcccttctcctccgggctgtaattagctgagcaagaggtaagggtttaagggatggttggttggtggggtattaatgtttaattacctggagcacctgcctgaaatcactttttttcaggtacacccaagctgtctagagccgccacc

SEQ ID NO: 24 - DNA, 7226 bp, synthetic construct
  source 1..7226: mol_type = other DNA
cacctaaattgtaagcgttaatattttgttaaaattcgcgttaaatttttgttaaatcagctcattttttaaccaataggccgaaatcggcaaaatcccttataaatcaaaagaatagaccgagatagggttgagtgttgttccagtttggaacaagagtccactattaaagaacgtggactccaacgtcaaagggcgaaaaaccgtctatcagggcgatggcccactacgtgaaccatcaccctaatcaagttttttggggtcgaggtgccgtaaagcactaaatcggaaccctaaagggagcccccgatttagagcttgacggggaaagccggcgaacgtggcgagaaaggaagggaagaaagcgaaaggagcgggcgctagggcgctggcaagtgtagcggtcacgctgcgcgtaaccaccacacccgccgcgcttaatgcgccgctacagggcgcgtcccattcgccattcaggctgcgcaactgttgggaagggcgatcggtgcgggcctcttcgctattacgccagctggcgaaagggggatgtgctgcaaggcgattaagttgggtaacgccagggttttcccagtcacgacgttgtaaaacgacggccagtgaattgtaatacgactcactatagggcgaattggagctccaccgcggtggcggccgctctagagtcctgtattagaggtcacgtgagtgttttgcgacattttgcgacaccatgtggtcacgctgggtatttaagcccgagtgagcacgcagggtctccattttgaagcgggaggtttgaacgcgcagccaccacggcggggttttacgagattgtgattaaggtccccagcgaccttgacgggcatctgcccggcatttctgacagctttgtgaactgggtggccgagaaggaatgggagttgccgccagattctgacatggatctgaatctgattgagcaggcacccctgaccgtggccgagaagctgcagcgcgactttctgacggaatggcgccgtgtgagtaaggccccggaggcccttttctttgtgcaatttgagaagggagagagctacttccacatgcacgtgctcgtggaaaccaccggggtgaaatccatggttttgggacgtttcctgagtcagattcgcgaaaaactgattcagagaatttaccgcgggatcgagccgactttgccaaactggttcgcggtcacaaagaccagaaatggcgccggaggcgggaacaaggtggtggatgagtgctacatccccaattacttgctccccaaaacccagcctgagctccagtgggcgtggactaatatggaacagtatttaagcgcctgtttgaatctcacggagcgtaaacggttggtggcgcagcatctgacgcacgtgtcgcagacgcaggagcagaacaaagagaatcagaatcccaattctgatgcgccggtgatcagatcaaaaacttcagccaggtacatggagctggtcgggtggctcgtggacaaggggattacctcggagaagcagtggatccaggaggaccaggcctcatacatctccttcaatgcggcctccaactcgcggtcccaaatcaaggctgccttggacaatgcgggaaagattatgagcctgactaaaaccgcccccgactacctggtgggccagcagcccgtggaggacatttccagcaatcggatttataaaattttggaactaaacgggtacgatccccaatatgcggcttccgtctttctgggatgggccacgaaaaagttcggcaagaggaacaccatctggctgtttgggcctgcaactaccgggaagaccaacatcgcggaggccatagcccacactgtgcccttctacgggtgcgtaaactggaccaatgagaactttcccttcaacgactgtgtcgacaagatggtgatctggtgggaggaggggaagatgaccgccaaggtcgtggagtcggccaaagccattctcggaggaagcaaggtgcgcgtggaccagaaatgcaagtcctcggcccagatagacccgactcccgtgatcgtcacctccaacaccaacatgtgcgccgtgattgacgggaactcaacgaccttcgaacaccagcagccgttgcaagaccggatgttcaaatttgaactcacccgccgtctggatcatgactttgggaaggtcaccaagcaggaagtcaaagactttttccggtgggcaaaggatcacgtggttgaggtggagcatgaattctacgtcaaaaagggtggagccaagaaaagacccgcccccagtgacgcagatataagtgagcccaaacgggtgcgcgagtcagttgcgcagccatcgacgtcagacgcggaagcttcgatcaactacgcagacaggtaccaaaacaaatgttctcgtcacgtgggcatgaatctgatgctgtttccctgcagacaatgcgagagaatgaatcagaattcaaatatctgcttcactcacggacagaaagactgtttagagtgctttcccgtgtcagaatctcaacccgtttctgtcgtcaaaaaggcgtatcagaaactgtgctacattcatcatatcatgggaaaggtgccagacgcttgcactgcctgcgatctggtcaatgtggatttggatgactgcatctttgaacaataaatgatttaaatagtcatgtcttttgttgatcaccctccagattggttggaagaagttggtgaaggtcttcgcgagtttttgggccttgaagcgggcccaccgaaaccaaaacccaatcagcagcatcaagatcaagcccgtggtcttgtgctgcctggttataactatctcggacccggaaacggtctcgatcgaggagagcctgtcaacagggcagacgaggtcgcgcgagagcacgacatctcgtacaacgagcagcttgaggcgggagacaacccctacctcaagtacaaccacgcggacgccgagtttcaggagaagctcgccgacgacacatccttcgggggaaacctcggaaaggcagtctttcaggccaagaaaagggttctcgaaccttttggcctggttgaagagggtgctaagacggcccctaccggaaagcggatagacgaccactttccaaaaagaaagaaggctcggaccgaagaggactccaagccttccacctcgtcagacgccgaagctggacccagcggatcccagcagctgcaaatcccagcccaaccagcctcaagtttgggagctgatacaatgtctgcgggaggtggcggcccattgggcgacaataaccaaggtgccgatggagtgggcaatgcctcgggagattggcattgcgattccacgtggatgggggacagagtcgtcaccaagtccacccgaacctgggtgctgcccagctacaacaaccaccagtaccgagagatcaaaagcggctccgtcgacggaagcaacgccaacgcctactttggatacagcaccccctgggggtactttgactttaaccgcttccacagccactggagcccccgagactggcaaagactcatcaacaactactggggcttcagaccccggtccctcagagtcaaaatcttcaacattcaagtcaaagaggtcacggtgcaggactccaccaccaccatcgccaacaacctcacctccaccgtccaagtgtttacggacgacgactaccagctgccctacgtcgtcggcaacgggaccgagggatgcctgccggccttccctccgcaggtctttacgctgccgcagtacggttacgcgacgctgaaccgcgacaacacagaaaatcccaccgagaggagcagcttcttctgcctagagtactttcccagcaagatgctgagaacgggcaacaactttgagtttacctacaactttgaggaggtgcccttccactccagcttcgctcccagtcagaacctgttcaagctggccaacccgctggtggaccagtacttgtaccgcttcgtgagcacaaataacactggcggagtccagttcaacaagaacctggccgggagatacgccaacacctacaaaaactggttcccggggcccatgggccgaacccagggctggaacctgggctccggggtcaaccgcgccagtgtcagcgccttcgccacgaccaataggatggagctcgagggcgcgagttaccaggtgcccccgcagccgaacggcatgaccaacaacctccagggcagcaacacctatgccctggagaacactatgatcttcaacagccagccggcgaacccgggcaccaccgccacgtacctcgagggcaacatgctcatcaccagcgagagcgagacgcagccggtgaaccgcgtggcgtacaacgtcggcgggcagatggccaccaacaaccagagctccaccactgcccccgcgaccggcacgtacaacctccaggaaatcgtgcccggcagcgtgtggatggagagggacgtgtacctccaaggacccatctgggccaagatcccagagacgggggcgcactttcacccctctccggccatgggcggattcggactcaaacacccaccgcccatgatgctcatcaagaacacgcctgtgcccggaaatatcaccagcttctcggacgtgcccgtcagcagcttcatcacccagtacagcaccgggcaggtcaccgtggagatggagtgggagctcaagaaggaaaactccaagaggtggaacccagagatccagtacacaaacaactacaacgacccccagtttgtggactttgccccggacagcaccggggaatacagaaccaccagacctatcggaacccgataccttacccgacccctttaacccattcatgtcgcataccctcaataaaccgtgtattcgtgtcagtaaaatactgcctcttgtggtcatttctagaactagaactagtggatcccccgggctgcaggaattcgatatcaagcttatcgataccgtcgacctcgagggggggcccggtacccagcttttgttccctttagtgagggttaatttcgagcttggcgtaatcatggtcatagctgtttcctgtgtgaaattgttatccgctcacaattccacacaacatacgagccggaagcataaagtgtaaagcctggggtgcctaatgagtgagctaactcacattaattgcgttgcgctcactgcccgctttccagtcgggaaacctgtcgtgccagctgcattaatgaatcggccaacgcgcggggagaggcggtttgcgtattgggcgctcttccgcttcctcgctcactgactcgctgcgctcggtcgttcggctgcggcgagcggtatcagctcactcaaaggcggtaatacggttatccacagaatcaggggataacgcaggaaagaacatgtgagcaaaaggccagcaaaaggccaggaaccgtaaaaaggccgcgttgctggcgtttttccataggctccgcccccctgacgagcatcacaaaaatcgacgctcaagtcagaggtggcgaaacccgacaggactataaagataccaggcgtttccccctggaagctccctcgtgcgctctcctgttccgaccctgccgcttaccggatacctgtccgcctttctcccttcgggaagcgtggcgctttctcatagctcacgctgtaggtatctcagttcggtgtaggtcgttcgctccaagctgggctgtgtgcacgaaccccccgttcagcccgaccgctgcgccttatccggtaactatcgtcttgagtccaacccggtaagacacgacttatcgccactggcagcagccactggtaacaggattagcagagcgaggtatgtaggcggtgctacagagttcttgaagtggtggcctaactacggctacactagaaggacagtatttggtatctgcgctctgctgaagccagttaccttcggaaaaagagttggtagctcttgatccggcaaacaaaccaccgctggtagcggtggtttttttgtttgcaagcagcagattacgcgcagaaaaaaaggatctcaagaagatcctttgatcttttctacggggtctgacgctcagtggaacgaaaactcacgttaagggattttggtcatgagattatcaaaaaggatcttcacctagatccttttaaattaaaaatgaagttttaaatcaatctaaagtatatatgagtaaacttggtctgacagttaccaatgcttaatcagtgaggcacctatctcagcgatctgtctatttcgttcatccatagttgcctgactccccgtcgtgtagataactacgatacgggagggcttaccatctggccccagtgctgcaatgataccgcgagacccacgctcaccggctccagatttatcagcaataaaccagccagccggaagggccgagcgcagaagtggtcctgcaactttatccgcctccatccagtctattaattgttgccgggaagctagagtaagtagttcgccagttaatagtttgcgcaacgttgttgccattgctacaggcatcgtggtgtcacgctcgtcgtttggtatggcttcattcagctccggttcccaacgatcaaggcgagttacatgatcccccatgttgtgcaaaaaagcggttagctccttcggtcctccgatcgttgtcagaagtaagttggccgcagtgttatcactcatggttatggcagcactgcataattctcttactgtcatgccatccgtaagatgcttttctgtgactggtgagtactcaaccaagtcattctgagaatagtgtatgcggcgaccgagttgctcttgcccggcgtcaatacgggataataccgcgccacatagcagaactttaaaagtgctcatcattggaaaacgttcttcggggcgaaaactctcaaggatcttaccgctgttgagatccagttcgatgtaacccactcgtgcacccaactgatcttcagcatcttttactttcaccagcgtttctgggtgagcaaaaacaggaaggcaaaatgccgcaaaaaagggaataagggcgacacggaaatgttgaatactcatactcttcctttttcaatattattgaagcatttatcagggttattgtctcatgagcggatacatatttgaatgtatttagaaaaataaacaaataggggttccgcgcacatttccccgaaaagtgc

SEQ ID NO: 25 - DNA, 7331 bp, synthetic construct
  source 1..7331: mol_type = other DNA
cccattcgccattcaggctgcgcaactgttgggaagggcgatcggtgcgggcctcttcgctattacgccagctggcgaaagggggatgtgctgcaaggcgattaagttgggtaacgccagggttttcccagtcacgacgttgtaaaacgacggccagtgagcgcgcgtaatacgactcactatagggcgaattgggtaccgggccccccctcgatcgaggtcgacggtatcgggggagctcgcagggtctccattttgaagcgggaggtttgaacgcgcagccgccatgccggggttttacgagattgtgattaaggtccccagcgaccttgacgagcatctgcccggcatttctgacagctttgtgaactgggtggccgagaaggaatgggagttgccgccagattctgacatggatctgaatctgattgagcaggcacccctgaccgtggccgagaagctgcagcgcgactttctgacggaatggcgccgtgtgagtaaggccccggaggctcttttctttgtgcaatttgagaagggagagagctacttccacatgcacgtgctcgtggaaaccaccggggtgaaatccatggttttgggacgtttcctgagtcagattcgcgaaaaactgattcagagaatttaccgcgggatcgagccgactttgccaaactggttcgcggtcacaaagaccagaaatggcgccggaggcgggaacaaggtggtggatgagtgctacatccccaattacttgctccccaaaacccagcctgagctccagtgggcgtggactaatatggaacagtatttaagcgcctgtttgaatctcacggagcgtaaacggttggtggcgcagcatctgacgcacgtgtcgcagacgcaggagcagaacaaagagaatcagaatcccaattctgatgcgccggtgatcagatcaaaaacttcagccaggtacatggagctggtcgggtggctcgtggacaaggggattacctcggagaagcagtggatccaggaggaccaggcctcatacatctccttcaatgcggcctccaactcgcggtcccaaatcaaggctgccttggacaatgcgggaaagattatgagcctgactaaaaccgcccccgactacctggtgggccagcagcccgtggaggacatttccagcaatcggatttataaaattttggaactaaacgggtacgatccccaatatgcggcttccgtctttctgggatgggccacgaaaaagttcggcaagaggaacaccatctggctgtttgggcctgcaactaccgggaagaccaacatcgcggaggccatagcccacactgtgcccttctacgggtgcgtaaactggaccaatgagaactttcccttcaacgactgtgtcgacaagatggtgatctggtgggaggaggggaagatgaccgccaaggtcgtggagtcggccaaagccattctcggaggaagcaaggtgcgcgtggaccagaaatgcaagtcctcggcccagatagacccgactcccgtgatcgtcacctccaacaccaacatgtgcgccgtgattgacgggaactcaacgaccttcgaacaccagcagccgttgcaagaccggatgttcaaatttgaactcacccgccgtctggatcatgactttgggaaggtcaccaagcaggaagtcaaagactttttccggtgggcaaaggatcacgtggttgaggtggagcatgaattctacgtcaaaaagggtggagccaagaaaagacccgcccccagtgacgcagatataagtgagcccaaacgggtgcgcgagtcagttgcgcagccatcgacgtcagacgcggaagcttcgatcaactacgcggacaggtaccaaaacaaatgttctcgtcacgtgggcatgaatctgatgctgtttccctgcagacaatgcgagagactgaatcagaattcaaatatctgcttcactcacggtgtcaaagactgtttagagtgctttcccgtgtcagaatctcaacccgtttctgtcgtcaaaaaggcgtatcagaaactgtgctacattcatcacatcatgggaaaggtgccagacgcttgcactgcttgcgacctggtcaatgtggacttggatgactgtgtttctgaacaataaatgacttaaaccaggtatggctgccgatggttatcttccagattggctcgaggacaaccttagtgaaggaattcgcgagtggtgggctttgaaacctggagcccctcaacccaaggcaaatcaacaacatcaagacaacgctcgaggtcttgtgcttccgggttacaaataccttggacccggcaacggactcgacaagggggagccggtcaacgcagcagacgcggcggccctcgagcacgacaaggcctacgaccagcagctcaaggccggagacaacccgtacctcaagtacaaccacgccgacgccgagttccaggagcggctcaaagaagatacgtcttttgggggcaacctcgggcgagcagtcttccaggccaaaaagaggcttcttgaacctcttggtctggttgaggaagcggctaagacggctcctggaaagaagaggcctgtagagcagtctcctcaggaaccggactcctccgcgggtattggcaaatcgggtgcacagcccgctaaaaagagactcaatttcggtcagactggcgacacagagtcagtcccagaccctcaaccaatcggagaacctcccgcagccccctcaggtgtgggatctcttacaatggcttcaggtggtggcgcaccagtggcagacaataacgaaggtgccgatggagtgggtagttcctcgggaaattggcattgcgattcccaatggctgggggacagagtcatcaccaccagcacccgaacctgggccctgcccacctacaacaatcacctctacaagcaaatctccaacagcacatctggaggatcttcaaatgacaacgcctacttcggctacagcaccccctgggggtattttgacttcaacagattccactgccacttctcaccacgtgactggcagcgactcatcaacaacaactggggattccggcctaagcgactcaacttcaagctcttcaacattcaggtcaaagaggttacggacaacaatggagtcaagaccatcgccaataaccttaccagcacggtccaggtcttcacggactcagactatcagctcccgtacgtgctcgggtcggctcacgagggctgcctcccgccgttcccagcggacgttttcatgattcctcagtacgggtatctgacgcttaatgatggaagccaggccgtgggtcgttcgtccttttactgcctggaatatttcccgtcgcaaatgctaagaacgggtaacaacttccagttcagctacgagtttgagaacgtacctttccatagcagctacgctcacagccaaagcctggaccgactaatgaatccactcatcgaccaatacttgtactatctctcaaagactattaacggttctggacagaatcaacaaacgctaaaattcagtgtggccggacccagcaacatggctgtccagggaagaaactacatacctggacccagctaccgacaacaacgtgtctcaaccactgtgactcaaaacaacaacagcgaatttgcttggcctggagcttcttcttgggctctcaatggacgtaatagcttgatgaatcctggacctgctatggccagccacaaagaaggagaggaccgtttctttcctttgtctggatctttaatttttggcaaacaaggaactggaagagacaacgtggatgcggacaaagtcatgataaccaacgaagaagaaattaaaactactaacccggtagcaacggagtcctatggacaagtggccacaaaccaccagagtgcccaagcacaggcgcagaccggctgggttcaaaaccaaggaatacttccgggtatggtttggcaggacagagatgtgtacctgcaaggacccatttgggccaaaattcctcacacggacggcaactttcacccttctccgctgatgggagggtttggaatgaagcacccgcctcctcagatcctcatcaaaaacacacctgtacctgcggatcctccaacggccttcaacaaggacaagctgaactctttcatcacccagtattctactggccaagtcagcgtggagatcgagtgggagctgcagaaggaaaacagcaagcgctggaacccggagatccagtacacttccaactattacaagtctaataatgttgaatttgctgttaatactgaaggtgtatatagtgaaccccgccccattggcaccagatacctgactcgtaatctgtaattgcttgttaatcaataaaccgtttaattcgtttcagttgaactttggtctctgcgaagggcgaattcgtttaaacctgcaggactagaggtcctgtattagaggtcacgtgagtgttttgcgacattttgcgacaccatgtggtcacgctgggtatttaagcccgagtgagcacgcagggtctccattttgaagcgggaggtttgaacgcgcagccgccaagccgaattctgcagatatccatcacactggcggccgctcgactagagcggccgccaccgcggtggagctccagcttttgttccctttagtgagggttaattgcgcgcttggcgtaatcatggtcatagctgtttcctgtgtgaaattgttatccgctcacaattccacacaacatacgagccggaagcataaagtgtaaagcctggggtgcctaatgagtgagctaactcacattaattgcgttgcgctcactgcccgctttccagtcgggaaacctgtcgtgccagctgcattaatgaatcggccaacgcgcggggagaggcggtttgcgtattgggcgctcttccgcttcctcgctcactgactcgctgcgctcggtcgttcggctgcggcgagcggtatcagctcactcaaaggcggtaatacggttatccacagaatcaggggataacggcaggaaagaacatgtgagcaaaaggccagcaaaaggccaggaaccgtaaaaaggccgcgttgctggcgtttttccataggctccgcccccctgacgagcatcacaaaaatcgacgctcaagtcagaggtggcgaaacccgacaggactataaagataccaggcgtttccccctggaagctccctcgtgcgctctcctgttccgaccctgccgcttaccggatacctgtccgcctttctcccttcgggaagcgtggcgctttctcatagctcacgctgtaggtatctcagttcggtgtaggtcgttcgctccaagctgggctgtgtgcacgaaccccccgttcagcccgaccgctgcgccttatccggtaactatcgtcttgagtccaacccggtaagacacgacttatcgccactggcagcagccactggtaacaggattagcagagcgaggtatgtaggcggtgctacagagttcttgaagtggtggcctaactacggctacactagaagaacagtatttggtatctgcgctctgctgaagccagttaccttcggaaaaagagttggtagctcttgatccggcaaacaaaccaccgctggtagcggtggtttttttgtttgcaagcagcagattacgcgcagaaaaaaaggatctcaagaagatcctttgatcttttctacggggtctgacgctcagtggaacgaaaactcacgttaagggattttggtcatgagattatcaaaaaggatcttcacctagatccttttaaattaaaaatgaagttttaaatcaatctaaagtatatatgagtaaacttggtctgacagttaccaatgcttaatcagtgaggcacctatctcagcgatctgtctatttcgttcatccatagttgcctgactccccgtcgtgtagataactacgatacgggagggcttaccatctggccccagtgctgcaatgataccgcgagacccacgctcaccggctccagatttatcagcaataaaccagccagccggaagggccgagcgcagaagtggtcctgcaactttatccgcctccatccagtctattaattgttgccgggaagctagagtaagtagttcgccagttaatagtttgcgcaacgttgttgccattgctacaggcatcgtggtgtcacgctcgtcgtttggtatggcttcattcagctccggttcccaacgatcaaggcgagttacatgatcccccatgttgtgcaaaaaagcggttagctccttcggtcctccgatcgttgtcagaagtaagttggccgcagtgttatcactcatggttatggcagcactgcataattctcttactgtcatgccatccgtaagatgcttttctgtgactggtgagtactcaaccaagtcattctgagaatagtgtatgcggcgaccgagttgctcttgcccggcgtcaatacgggataataccgcgccacatagcagaactttaaaagtgctcatcattggaaaacgttcttcggggcgaaaactctcaaggatcttaccgctgttgagatccagttcgatgtaacccactcgtgcacccaactgatcttcagcatcttttactttcaccagcgtttctgggtgagcaaaaacaggaaggcaaaatgccgcaaaaaagggaataagggcgacacggaaatgttgaatactcatactcttcctttttcaatattattgaagcatttatcagggttattgtctcatgagcggatacatatttgaatgtatttagaaaaataaacaaataggggttccgcgcacatttccccgaaaagtgccacctaaattgtaagcgttaatattttgttaaaattcgcgttaaatttttgttaaatcagctcattttttaaccaataggccgaaatcggcaaaatcccttataaatcaaaagaatagaccgagatagggttgagtgttgttccagtttggaacaagagtccactattaaagaacgtggactccaacgtcaaagggcgaaaaaccgtctatcagggcgatggcccactacgtgaaccatcaccctaatcaagttttttggggtcgaggtgccgtaaagcactaaatcggaaccctaaagggagcccccgatttagagcttgacggggaaagccggcgaacgtggcgagaaaggaagggaagaaagcgaaaggagcgggcgctagggcgctggcaagtgtagcggtcacgctgcgcgtaaccaccacacccgccgcgcttaatgcgccgctacagggcgcgt

SEQ ID NO: 26 - DNA, 8543 bp, synthetic construct
  source 1..8543: mol_type = other DNA
ccaatgatacgcgtcggtgcgggcctcttcgctattacgccagctggcgaaagggggatgtgctgcaaggcgattaagttgggtaacgccagggttttcccagtcacgacgttgtaaaacgacggccagtgagcgcgcgtaatacgactcactatagggcgaattgggtacatcgacggtatcgggggagctcgcagggtctccattttgaagcgggaggtttgaacgcgcagccgccatgccggggttttacgagattgtgattaaggtccccagcgaccttgacgagcatctgcccggcatttctgacagctttgtgaactgggtggccgagaaggaatgggagttgccgccagattctgacatggatctgaatctgattgagcaggcacccctgaccgtggccgagaagctgcagcgcgactttctgacggaatggcgccgtgtgagtaaggccccggaggctcttttctttgtgcaatttgagaagggagagagctacttccacatgcacgtgctcgtggaaaccaccggggtgaaatccatggttttgggacgtttcctgagtcagattcgcgaaaaactgattcagagaatttaccgcgggatcgagccgactttgccaaactggttcgcggtcacaaagaccagaaatggcgccggaggcgggaacaaggtggtggatgagtgctacatccccaattacttgctccccaaaacccagcctgagctccagtgggcgtggactaatatggaacagtatttaagcgcctgtttgaatctcacggagcgtaaacggttggtggcgcagcatctgacgcacgtgtcgcagacgcaggagcagaacaaagagaatcagaatcccaattctgatgcgccggtgatcagatcaaaaacttcagccaggtacatggagctggtcgggtggctcgtggacaaggggattacctcggagaagcagtggatccaggaggaccaggcctcatacatctccttcaatgcggcctccaactcgcggtcccaaatcaaggctgccttggacaatgcgggaaagattatgagcctgactaaaaccgcccccgactacctggtgggccagcagcccgtggaggacatttccagcaatcggatttataaaattttggaactaaacgggtacgatccccaatatgcggcttccgtctttctgggatgggccacgaaaaagttcggcaagaggaacaccatctggctgtttgggcctgcaactaccgggaagaccaacatcgcggaggccatagcccacactgtgcccttctacgggtgcgtaaactggaccaatgagaactttcccttcaacgactgtgtggacaagatggtgatctggtgggaggaggggaagatgaccgccaaggtcgtggagtcggccaaagccattctcggaggaagcaaggtgcgcgtggaccagaaatgcaagtcctcggcccagatagacccgactcccgtgatcgtcacctccaacaccaatatgtgcgccgtgattgacgggaactcaacgaccttcgaacaccagcagccgttgcaagaccggatgttcaaatttgaactcacccgccgtctggatcatgactttgggaaggtcaccaagcaggaagtcaaagactttttccggtgggcaaaggatcacgtggttgaggtggagcatgaattctacgtcaaaaagggtggagccaagaaaagacccgcccccagtgacgcagatataagtgagcccaaacgggtgcgcgagtcagttgcgcagccatcgacgtcagacgcggaagcttcgatcaactacgcggacaggtaccaaaacaaatgttctcgtcacgtgggcatgaatctgatgctgtttccctgcagacaatgcgagagactgaatcagaattcaaatatctgcttcactcacggtgtcaaagactgtttagagtgctttcccgtgtcagaatctcaacccgtttctgtcgtcaaaaaggcgtatcagaaactgtgctacattcatcacatcatgggaaaggtgccagacgcttgcactgcttgcgacctggtcaatgtggacttggatgactgtgtttctgaacaataaatgacttaaaccaggtatgagtcggctggataaatctaaagtcataaacggcgctctggaattactcaatgaagtcggtatcgaaggcctgacgacaaggaaactcgctcaaaagctgggagttgagcagcctaccctgtactggcacgtgaagaacaagcgggccctgctcgatgccctggccatcgagatgctggacaggcatcatacccacttctgccccctggaaggcgagtcatggcaagactttctgcggaacaacgccaagtcattccgctgtgctctcctctcacatcgcgacggggctaaagtgcatctcggcacccgcccaacagagaaacagtacgaaaccctggaaaatcagctcgcgttcctgtgtcagcaaggcttctccctggagaacgcactgtacgctctgtccgccgtgggccactttacactgggctgcgtattggaggaacaggagcatcaagtagcaaaagaggaaagagagacacctaccaccgattctatgcccccacttctgagacaagcaattgagctgttcgaccggcagggagccgaacctgccttccttttcggcctggaactaatcatatgtggcctggagaaacagctaaagtgcgaaagcggcgggccggccgacgcccttgacgattttgacttagacatgctcccagccgatgcccttgacgactttgaccttgatatgctgcctgctgacgctcttgacgattttgaccttgacatgctccccgggtaaatgcatgaattcgatctagagggccctattctatagtgtcacctaaatgctagagctcgctgatcagcctcgactgtgccttctagttgccagccatctgttgtttgcccctcccccgtgccttccttgaccctggaaggtgccactcccactgtcctttcctaataaaatgaggaaattgcatcgcattgtctgagtaggtgtcattctattctggggggtggggtggggcaggacagcaagggggaggattgggaagacaatagcaggcatgctggggatgcggtgggctctatggcttctgaggcggaaagaaccagctggggctcgaatcaagctatcaagtgccacctgacgtctccctatcagtgatagagaagtcgacacgtctcgagctccctatcagtgatagagaaggtacgtctagaacgtctccctatcagtgatagagaagtcgacacgtctcgagctccctatcagtgatagagaaggtacgtctagaacgtctccctatcagtgatagagaagtcgacacgtctcgagctccctatcagtgatagagaaggtacgtctagaacgtctccctatcagtgatagagaagtcgacacgtctcgagctccctatcagtgatagagaaggtaccccctatataagcagagagatctgttcaaatttgaactgactaagcggctcccgccagattttggcaagattactaagcaggaagtcaaggacttttttgcttgggcaaaggtcaatcaggtgccggtgactcacgagtttaaagttcccagggaattggcgggaactaaaggggcggagaaatctctaaaacgcccactgggtgacgtcaccaatactagctataaaagtctggagaagcgggccaggctctcatttgttcccgagacgcctcgcagttcagacgtgactgttgatcccgctcctctgcgaccgctagcttcgatcaactacgcagacaggtaccaaaacaagtgttctcgtcacgtgggcattaatctgattctgtttccctgcagacaatgcgagagaatgaatcagaactcaaatatctgcttcactcacggacagaaagactgtttagagtgctttcccgtgtcagaatctcaacccgtttctgtcgtcaaaaaggcgtatcagaaactgtgctacattcatcatatcatgggaaaggtgccagacgcttgcactgcctgcgatctggtcaatgtggatttggatgactgcatctttgaacaataaatgacttaagccaggtatggctgccgatggttatcttccagattggctcgaggacaaccttagtgaaggaattcgcgagtggtgggctttgaaacctggagcccctcaacccaaggcaaatcaacaacatcaagacaacgctcgaggtcttgtgcttccgggttacaaataccttggacccggcaacggactcgacaagggggagccggtcaacgcagcagacgcggcggccctcgagcacgacaaggcctacgaccagcagctcaaggccggagacaacccgtacctcaagtacaaccacgccgacgccgagttccaggagcggctcaaagaagatacgtcttttgggggcaacctcgggcgagcagtcttccaggccaaaaagaggcttcttgaacctcttggtctggttgaggaagcggctaagacggctcctggaaagaagaggcctgtagagcagtctcctcaggaaccggactcctccgcgggtattggcaaatcgggtgcacagcccgctaaaaagagactcaatttcggtcagactggcgacacagagtcagtcccagaccctcaaccaatcggagaacctcccgcagccccctcaggtgtgggatctcttacaatggcttcaggtggtggcgcaccagtggcagacaataacgaaggtgccgatggagtgggtagttcctcgggaaattggcattgcgattcccaatggctgggggacagagtcatcaccaccagcacccgaacctgggccctgcccacctacaacaatcacctctacaagcaaatctccaacagcacatctggaggatcttcaaatgacaacgcctacttcggctacagcaccccctgggggtattttgacttcaacagattccactgccacttctcaccacgtgactggcagcgactcatcaacaacaactggggattccggcctaagcgactcaacttcaagctcttcaacattcaggtcaaagaggttacggacaacaatggagtcaagaccatcgccaataaccttaccagcacggtccaggtcttcacggactcagactatcagctcccgtacgtgctcgggtcggctcacgagggctgcctcccgccgttcccagcggacgttttcatgattcctcagtacgggtatctgacgcttaatgatggaagccaggccgtgggtcgttcgtccttttactgcctggaatatttcccgtcgcaaatgctaagaacgggtaacaacttccagttcagctacgagtttgagaacgtacctttccatagcagctacgctcacagccaaagcctggaccgactaatgaatccactcatcgaccaatacttgtactatctctctagaactattaacggttctggacagaatcaacaaacgctaaaattcagtgtggccggacccagcaacatggctgtccagggaagaaactacatacctggacccagctaccgacaacaacgtgtctcaaccactgtgactcaaaacaacaacagcgaatttgcttggcctggagcttcttcttgggctctcaatggacgtaatagcttgatgaatcctggacctgctatggccagccacaaagaaggagaggaccgtttctttcctttgtctggatctttaatttttggcaaacaaggtaccggcagagacaacgtggatgcggacaaagtcatgataaccaacgaagaagaaattaaaactactaacccggtagcaacggagtcctatggacaagtggccacaaaccaccagagtgatgggactttggcggtgccttttaaggcacaggcgcagaccggttgggttcaaaaccaaggaatacttccgggtatggtttggcaggacagagatgtgtacctgcaaggacccatttgggccaaaattcctcacacggacggcaactttcacccttctccgctgatgggagggtttggaatgaagcacccgcctcctcagatcctcatcaaaaacacacctgtacctgcggatcctccaacggccttcaacaaggacaagctgaactctttcatcacccagtattctactggccaagtcagcgtggagatcgagtgggagctgcagaaggaaaacagcaagcgctggaacccggagatccagtacacttccaactattacaagtctaataatgttgaatttgctgttaatactgaaggtgtatatagtgaaccccgccccattggcaccagatacctgactcgtaatctgtaagtcgacttgcttgttaatcaataaaccgtttaattcgtttcagttgaactttggtctctgcgaagggcaattcgtttaaacctgcaggactagaggtcctgtattagaggtcacgtgagtgttttgcgacattttgcgacaccatgtggtcacgctgggtatttaagcccgagtgagcacgcagggtctccattttgaagcgggaggtttgaacgcgcagccgccaagccgaattctgcagatatcacatgtcctaggaactatcgatccatcacactggcggccgctcgactagagcggccgccaccgcggtggagctccagcttttgcggaccgaatcggaaagaacatgtgagcaaaaggccagcaaaaggccaggaaccgtaaaaaggccgcgttgctggcgtttttccataggctccgcccccctgacgagcatcacaaaaatcgacgctcaagtcagaggtggcgaaacccgacaggactataaagataccaggcgtttccccctggaagctccctcgtgcgctctcctgttccgaccctgccgcttaccggatacctgtccgcctttctcccttcgggaagcgtggcgctttctcatagctcacgctgtaggtatctcagttcggtgtaggtcgttcgctccaagctgggctgtgtgcacgaaccccccgttcagcccgaccgctgcgccttatccggtaactatcgtcttgagtccaacccggtaagacacgacttatcgccactggcagcagccactggtaacaggattagcagagcgaggtatgtaggcggtgctacagagttcttgaagtggtggcctaactacggctacactagaagaacagtatttggtatctgcgctctgctgaagccagttaccttcggaaaaagagttggtagctcttgatccggcaaacaaaccaccgctggtagcggtggtttttttgtttgcaagcagcagattacgcgcagaaaaaaaggatctcaagaagatcctttgatcttttctacggggtctgacgctcagtggaacgaaaactcacgttaagggattttggtcatgagattatcaaaaaggatcttcacctagatccttttaaattaaaaatgaagttttaaatcaatctaaagtatatatgagtaaacttggtctgacagttaccaatgcttaatcagtgaggcacctatctcagcgatctgtctatttcgttcatccatagttgcctgactccccgtcgtgtagataactacgatacgggagggcttaccatctggccccagtgctgcaatgataccgcgagacccacgctcaccggctccagatttatcagcaataaaccagccagccggaagggccgagcgcagaagtggtcctgcaactttatccgcctccatccagtctattaattgttgccgggaagctagagtaagtagttcgccagttaatagtttgcgcaacgttgttgccattgctacaggcatcgtggtgtcacgctcgtcgtttggtatggcttcattcagctccggttcccaacgatcaaggcgagttacatgatcccccatgttgtgcaaaaaagcggttagctccttcggtcctccgatcgttgtcagaagtaagttggccgcagtgttatcactcatggttatggcagcactgcataattctcttactgtcatgccatccgtaagatgcttttctgtgactggtgagtactcaaccaagtcattctgagaatagtgtatgcggcgaccgagttgctcttgcccggcgtcaatacgggataataccgcgccacatagcagaactttaaaagtgctcatcattggaaaacgttcttcggggcgaaaactctcaaggatcttaccgctgttgagatccagttcgatgtaacccactcgtgcacccaactgatcttcagcatcttttactttcaccagcgtttctgggtgagcaaaaacaggaaggcaaaatgccgcaaaaaagggaataagggcgacacggaaatgttgaatactcatactcttcctttttcaatattattgaagcatttatcagggttattgtctcatgagcggatacatatttgaatgtatttagaaaaataaacaaataggggttccgcgcacatttccccgaaaagtgccacctgacgtc

SEQ ID NO: 27 - DNA, 8543 bp, synthetic construct
  source 1..8543: mol_type = other DNA
ccaatgatacgcgtcggtgcgggcctcttcgctattacgccagctggcgaaagggggatgtgctgcaaggcgattaagttgggtaacgccagggttttcccagtcacgacgttgtaaaacgacggccagtgagcgcgcgtaatacgactcactatagggcgaattgggtacatcgacggtatcgggggagctcgcagggtctccattttgaagcgggaggtttgaacgcgcagccgccatgccggggttttacgagattgtgattaaggtccccagcgaccttgacgagcatctgcccggcatttctgacagctttgtgaactgggtggccgagaaggaatgggagttgccgccagattctgacatggatctgaatctgattgagcaggcacccctgaccgtggccgagaagctgcagcgcgactttctgacggaatggcgccgtgtgagtaaggccccggaggctcttttctttgtgcaatttgagaagggagagagctacttccacatgcacgtgctcgtggaaaccaccggggtgaaatccatggttttgggacgtttcctgagtcagattcgcgaaaaactgattcagagaatttaccgcgggatcgagccgactttgccaaactggttcgcggtcacaaagaccagaaatggcgccggaggcgggaacaaggtggtggatgagtgctacatccccaattacttgctccccaaaacccagcctgagctccagtgggcgtggactaatatggaacagtatttaagcgcctgtttgaatctcacggagcgtaaacggttggtggcgcagcatctgacgcacgtgtcgcagacgcaggagcagaacaaagagaatcagaatcccaattctgatgcgccggtgatcagatcaaaaacttcagccaggtacatggagctggtcgggtggctcgtggacaaggggattacctcggagaagcagtggatccaggaggaccaggcctcatacatctccttcaatgcggcctccaactcgcggtcccaaatcaaggctgccttggacaatgcgggaaagattatgagcctgactaaaaccgcccccgactacctggtgggccagcagcccgtggaggacatttccagcaatcggatttataaaattttggaactaaacgggtacgatccccaatatgcggcttccgtctttctgggatgggccacgaaaaagttcggcaagaggaacaccatctggctgtttgggcctgcaactaccgggaagaccaacatcgcggaggccatagcccacactgtgcccttctacgggtgcgtaaactggaccaatgagaactttcccttcaacgactgtgtggacaagatggtgatctggtgggaggaggggaagatgaccgccaaggtcgtggagtcggccaaagccattctcggaggaagcaaggtgcgcgtggaccagaaatgcaagtcctcggcccagatagacccgactcccgtgatcgtcacctccaacaccaatatgtgcgccgtgattgacgggaactcaacgaccttcgaacaccagcagccgttgcaagaccggatgttcaaatttgaactcacccgccgtctggatcatgactttgggaaggtcaccaagcaggaagtcaaagactttttccggtgggcaaaggatcacgtggttgaggtggagcatgaattctacgtcaaaaagggtggagccaagaaaagacccgcccccagtgacgcagatataagtgagcccaaacgggtgcgcgagtcagttgcgcagccatcgacgtcagacgcggaagcttcgatcaactacgcggacaggtaccaaaacaaatgttctcgtcacgtgggcatgaatctgatgctgtttccctgcagacaatgcgagagactgaatcagaattcaaatatctgcttcactcacggtgtcaaagactgtttagagtgctttcccgtgtcagaatctcaacccgtttctgtcgtcaaaaaggcgtatcagaaactgtgctacattcatcacatcatgggaaaggtgccagacgcttgcactgcttgcgacctggtcaatgtggacttggatgactgtgtttctgaacaataaatgacttaaaccaggtatgagtcggctggataaatctaaagtcataaacggcgctctggaattactcaatgaagtcggtatcgaaggcctgacgacaaggaaactcgctcaaaagctgggagttgagcagcctaccctgtactggcacgtgaagaacaagcgggccctgctcgatgccctggccatcgagatgctggacaggcatcatacccacttctgccccctggaaggcgagtcatggcaagactttctgcggaacaacgccaagtcattccgctgtgctctcctctcacatcgcgacggggctaaagtgcatctcggcacccgcccaacagagaaacagtacgaaaccctggaaaatcagctcgcgttcctgtgtcagcaaggcttctccctggagaacgcactgtacgctctgtccgccgtgggccactttacactgggctgcgtattggaggaacaggagcatcaagtagcaaaagaggaaagagagacacctaccaccgattctatgcccccacttctgagacaagcaattgagctgttcgaccggcagggagccgaacctgccttccttttcggcctggaactaatcatatgtggcctggagaaacagctaaagtgcgaaagcggcgggccggccgacgcccttgacgattttgacttagacatgctcccagccgatgcccttgacgactttgaccttgatatgctgcctgctgacgctcttgacgattttgaccttgacatgctccccgggtaaatgcatgaattcgatctagagggccctattctatagtgtcacctaaatgctagagctcgctgatcagcctcgactgtgccttctagttgccagccatctgttgtttgcccctcccccgtgccttccttgaccctggaaggtgccactcccactgtcctttcctaataaaatgaggaaattgcatcgcattgtctgagtaggtgtcattctattctggggggtggggtggggcaggacagcaagggggaggattgggaagacaatagcaggcatgctggggatgcggtgggctctatggcttctgaggcggaaagaaccagctggggctcgaatcaagctatcaagtgccacctgacgtctccctatcagtgatagagaagtcgacacgtctcgagctccctatcagtgatagagaaggtacgtctagaacgtctccctatcagtgatagagaagtcgacacgtctcgagctccctatcagtgatagagaaggtacgtctagaacgtctccctatcagtgatagagaagtcgacacgtctcgagctccctatcagtgatagagaaggtacgtctagaacgtctccctatcagtgatagagaagtcgacacgtctcgagctccctatcagtgatagagaaggtaccccctatataagcagagagatctgttcaaatttgaactgactaagcggctcccgccagattttggcaagattactaagcaggaagtcaaggacttttttgcttgggcaaaggtcaatcaggtgccggtgactcacgagtttaaagttcccagggaattggcgggaactaaaggggcggagaaatctctaaaacgcccactgggtgacgtcaccaatactagctataaaagtctggagaagcgggccaggctctcatttgttcccgagacgcctcgcagttcagacgtgactgttgatcccgctcctctgcgaccgctagcttcgatcaactacgcagacaggtaccaaaacaagtgttctcgtcacgtgggcattaatctgattctgtttccctgcagacaatgcgagagaatgaatcagaactcaaatatctgcttcactcacggacagaaagactgtttagagtgctttcccgtgtcagaatctcaacccgtttctgtcgtcaaaaaggcgtatcagaaactgtgctacattcatcatatcatgggaaaggtgccagacgcttgcactgcctgcgatctggtcaatgtggatttggatgactgcatctttgaacaataaatgacttaagccaggtatggctgccgatggttatcttccagattggctcgaggacaaccttagtgaaggaattcgcgagtggtgggctttgaaacctggagcccctcaacccaaggcaaatcaacaacatcaagacaacgctcgaggtcttgtgcttccgggttacaaataccttggacccggcaacggactcgacaagggggagccggtcaacgcagcagacgcggcggccctcgagcacgacaaggcctacgaccagcagctcaaggccggagacaacccgtacctcaagtacaaccacgccgacgccgagttccaggagcggctcaaagaagatacgtcttttgggggcaacctcgggcgagcagtcttccaggccaaaaagaggcttcttgaacctcttggtctggttgaggaagcggctaagacggctcctggaaagaagaggcctgtagagcagtctcctcaggaaccggactcctccgcgggtattggcaaatcgggtgcacagcccgctaaaaagagactcaatttcggtcagactggcgacacagagtcagtcccagaccctcaaccaatcggagaacctcccgcagccccctcaggtgtgggatctcttacaatggcttcaggtggtggcgcaccagtggcagacaataacgaaggtgccgatggagtgggtagttcctcgggaaattggcattgcgattcccaatggctgggggacagagtcatcaccaccagcacccgaacctgggccctgcccacctacaacaatcacctctacaagcaaatctccaacagcacatctggaggatcttcaaatgacaacgcctacttcggctacagcaccccctgggggtattttgacttcaacagattccactgccacttctcaccacgtgactggcagcgactcatcaacaacaactggggattccggcctaagcgactcaacttcaagctcttcaacattcaggtcaaagaggttacggacaacaatggagtcaagaccatcgccaataaccttaccagcacggtccaggtcttcacggactcagactatcagctcccgtacgtgctcgggtcggctcacgagggctgcctcccgccgttcccagcggacgttttcatgattcctcagtacgggtatctgacgcttaatgatggaagccaggccgtgggtcgttcgtccttttactgcctggaatatttcccgtcgcaaatgctaagaacgggtaacaacttccagttcagctacgagtttgagaacgtacctttccatagcagctacgctcacagccaaagcctggaccgactaatgaatccactcatcgaccaatacttgtactatctctctagaactattaacggttctggacagaatcaacaaacgctaaaattcagtgtggccggacccagcaacatggctgtccagggaagaaactacatacctggacccagctaccgacaacaacgtgtctcaaccactgtgactcaaaacaacaacagcgaatttgcttggcctggagcttcttcttgggctctcaatggacgtaatagcttgatgaatcctggacctgctatggccagccacaaagaaggagaggaccgtttctttcctttgtctggatctttaatttttggcaaacaaggaactggaagagacaacgtggatgcggacaaagtcatgataaccaacgaagaagaaattaaaactactaacccggtagcaacggagtcctatggacaagtggccacaaaccaccagagtgcccaacaggcggttaggacgtctttggcacaggcgcagaccggttgggttcaaaaccaaggaatacttccgggtatggtttggcaggacagagatgtgtacctgcaaggacccatttgggccaaaattcctcacacggacggcaactttcacccttctccgctgatgggagggtttggaatgaagcacccgcctcctcagatcctcatcaaaaacacacctgtacctgcggatcctccaacggccttcaacaaggacaagctgaactctttcatcacccagtattctactggccaagtcagcgtggagatcgagtgggagctgcagaaggaaaacagcaagcgctggaacccggagatccagtacacttccaactattacaagtctaataatgttgaatttgctgttaatactgaaggtgtatatagtgaaccccgccccattggcaccagatacctgactcgtaatctgtaagtcgacttgcttgttaatcaataaaccgtttaattcgtttcagttgaactttggtctctgcgaagggcaattcgtttaaacctgcaggactagaggtcctgtattagaggtcacgtgagtgttttgcgacattttgcgacaccatgtggtcacgctgggtatttaagcccgagtgagcacgcagggtctccattttgaagcgggaggtttgaacgcgcagccgccaagccgaattctgcagatatcacatgtcctaggaactatcgatccatcacactggcggccgctcgactagagcggccgccaccgcggtggagctccagcttttgcggaccgaatcggaaagaacatgtgagcaaaaggccagcaaaaggccaggaaccgtaaaaaggccgcgttgctggcgtttttccataggctccgcccccctgacgagcatcacaaaaatcgacgctcaagtcagaggtggcgaaacccgacaggactataaagataccaggcgtttccccctggaagctccctcgtgcgctctcctgttccgaccctgccgcttaccggatacctgtccgcctttctcccttcgggaagcgtggcgctttctcatagctcacgctgtaggtatctcagttcggtgtaggtcgttcgctccaagctgggctgtgtgcacgaaccccccgttcagcccgaccgctgcgccttatccggtaactatcgtcttgagtccaacccggtaagacacgacttatcgccactggcagcagccactggtaacaggattagcagagcgaggtatgtaggcggtgctacagagttcttgaagtggtggcctaactacggctacactagaagaacagtatttggtatctgcgctctgctgaagccagttaccttcggaaaaagagttggtagctcttgatccggcaaacaaaccaccgctggtagcggtggtttttttgtttgcaagcagcagattacgcgcagaaaaaaaggatctcaagaagatcctttgatcttttctacggggtctgacgctcagtggaacgaaaactcacgttaagggattttggtcatgagattatcaaaaaggatcttcacctagatccttttaaattaaaaatgaagttttaaatcaatctaaagtatatatgagtaaacttggtctgacagttaccaatgcttaatcagtgaggcacctatctcagcgatctgtctatttcgttcatccatagttgcctgactccccgtcgtgtagataactacgatacgggagggcttaccatctggccccagtgctgcaatgataccgcgagacccacgctcaccggctccagatttatcagcaataaaccagccagccggaagggccgagcgcagaagtggtcctgcaactttatccgcctccatccagtctattaattgttgccgggaagctagagtaagtagttcgccagttaatagtttgcgcaacgttgttgccattgctacaggcatcgtggtgtcacgctcgtcgtttggtatggcttcattcagctccggttcccaacgatcaaggcgagttacatgatcccccatgttgtgcaaaaaagcggttagctccttcggtcctccgatcgttgtcagaagtaagttggccgcagtgttatcactcatggttatggcagcactgcataattctcttactgtcatgccatccgtaagatgcttttctgtgactggtgagtactcaaccaagtcattctgagaatagtgtatgcggcgaccgagttgctcttgcccggcgtcaatacgggataataccgcgccacatagcagaactttaaaagtgctcatcattggaaaacgttcttcggggcgaaaactctcaaggatcttaccgctgttgagatccagttcgatgtaacccactcgtgcacccaactgatcttcagcatcttttactttcaccagcgtttctgggtgagcaaaaacaggaaggcaaaatgccgcaaaaaagggaataagggcgacacggaaatgttgaatactcatactcttcctttttcaatattattgaagcatttatcagggttattgtctcatgagcggatacatatttgaatgtatttagaaaaataaacaaataggggttccgcgcacatttccccgaaaagtgccacctgacgtc

SEQ ID NO: 28 - DNA, 8543 bp, synthetic construct
  source 1..8543: mol_type = other DNA
ccaatgatacgcgtcggtgcgggcctcttcgctattacgccagctggcgaaagggggatgtgctgcaaggcgattaagttgggtaacgccagggttttcccagtcacgacgttgtaaaacgacggccagtgagcgcgcgtaatacgactcactatagggcgaattgggtacatcgacggtatcgggggagctcgcagggtctccattttgaagcgggaggtttgaacgcgcagccgccatgccggggttttacgagattgtgattaaggtccccagcgaccttgacgagcatctgcccggcatttctgacagctttgtgaactgggtggccgagaaggaatgggagttgccgccagattctgacatggatctgaatctgattgagcaggcacccctgaccgtggccgagaagctgcagcgcgactttctgacggaatggcgccgtgtgagtaaggccccggaggctcttttctttgtgcaatttgagaagggagagagctacttccacatgcacgtgctcgtggaaaccaccggggtgaaatccatggttttgggacgtttcctgagtcagattcgcgaaaaactgattcagagaatttaccgcgggatcgagccgactttgccaaactggttcgcggtcacaaagaccagaaatggcgccggaggcgggaacaaggtggtggatgagtgctacatccccaattacttgctccccaaaacccagcctgagctccagtgggcgtggactaatatggaacagtatttaagcgcctgtttgaatctcacggagcgtaaacggttggtggcgcagcatctgacgcacgtgtcgcagacgcaggagcagaacaaagagaatcagaatcccaattctgatgcgccggtgatcagatcaaaaacttcagccaggtacatggagctggtcgggtggctcgtggacaaggggattacctcggagaagcagtggatccaggaggaccaggcctcatacatctccttcaatgcggcctccaactcgcggtcccaaatcaaggctgccttggacaatgcgggaaagattatgagcctgactaaaaccgcccccgactacctggtgggccagcagcccgtggaggacatttccagcaatcggatttataaaattttggaactaaacgggtacgatccccaatatgcggcttccgtctttctgggatgggccacgaaaaagttcggcaagaggaacaccatctggctgtttgggcctgcaactaccgggaagaccaacatcgcggaggccatagcccacactgtgcccttctacgggtgcgtaaactggaccaatgagaactttcccttcaacgactgtgtggacaagatggtgatctggtgggaggaggggaagatgaccgccaaggtcgtggagtcggccaaagccattctcggaggaagcaaggtgcgcgtggaccagaaatgcaagtcctcggcccagatagacccgactcccgtgatcgtcacctccaacaccaatatgtgcgccgtgattgacgggaactcaacgaccttcgaacaccagcagccgttgcaagaccggatgttcaaatttgaactcacccgccgtctggatcatgactttgggaaggtcaccaagcaggaagtcaaagactttttccggtgggcaaaggatcacgtggttgaggtggagcatgaattctacgtcaaaaagggtggagccaagaaaagacccgcccccagtgacgcagatataagtgagcccaaacgggtgcgcgagtcagttgcgcagccatcgacgtcagacgcggaagcttcgatcaactacgcggacaggtaccaaaacaaatgttctcgtcacgtgggcatgaatctgatgctgtttccctgcagacaatgcgagagactgaatcagaattcaaatatctgcttcactcacggtgtcaaagactgtttagagtgctttcccgtgtcagaatctcaacccgtttctgtcgtcaaaaaggcgtatcagaaactgtgctacattcatcacatcatgggaaaggtgccagacgcttgcactgcttgcgacctggtcaatgtggacttggatgactgtgtttctgaacaataaatgacttaaaccaggtatgagtcggctggataaatctaaagtcataaacggcgctctggaattactcaatgaagtcggtatcgaaggcctgacgacaaggaaactcgctcaaaagctgggagttgagcagcctaccctgtactggcacgtgaagaacaagcgggccctgctcgatgccctggccatcgagatgctggacaggcatcatacccacttctgccccctggaaggcgagtcatggcaagactttctgcggaacaacgccaagtcattccgctgtgctctcctctcacatcgcgacggggctaaagtgcatctcggcacccgcccaacagagaaacagtacgaaaccctggaaaatcagctcgcgttcctgtgtcagcaaggcttctccctggagaacgcactgtacgctctgtccgccgtgggccactttacactgggctgcgtattggaggaacaggagcatcaagtagcaaaagaggaaagagagacacctaccaccgattctatgcccccacttctgagacaagcaattgagctgttcgaccggcagggagccgaacctgccttccttttcggcctggaactaatcatatgtggcctggagaaacagctaaagtgcgaaagcggcgggccggccgacgcccttgacgattttgacttagacatgctcccagccgatgcccttgacgactttgaccttgatatgctgcctgctgacgctcttgacgattttgaccttgacatgctccccgggtaaatgcatgaattcgatctagagggccctattctatagtgtcacctaaatgctagagctcgctgatcagcctcgactgtgccttctagttgccagccatctgttgtttgcccctcccccgtgccttccttgaccctggaaggtgccactcccactgtcctttcctaataaaatgaggaaattgcatcgcattgtctgagtaggtgtcattctattctggggggtggggtggggcaggacagcaagggggaggattgggaagacaatagcaggcatgctggggatgcggtgggctctatggcttctgaggcggaaagaaccagctggggctcgaatcaagctatcaagtgccacctgacgtctccctatcagtgatagagaagtcgacacgtctcgagctccctatcagtgatagagaaggtacgtctagaacgtctccctatcagtgatagagaagtcgacacgtctcgagctccctatcagtgatagagaaggtacgtctagaacgtctccctatcagtgatagagaagtcgacacgtctcgagctccctatcagtgatagagaaggtacgtctagaacgtctccctatcagtgatagagaagtcgacacgtctcgagctccctatcagtgatagagaaggtaccccctatataagcagagagatctgttcaaatttgaactgactaagcggctcccgccagattttggcaagattactaagcaggaagtcaaggacttttttgcttgggcaaaggtcaatcaggtgccggtgactcacgagtttaaagttcccagggaattggcgggaactaaaggggcggagaaatctctaaaacgcccactgggtgacgtcaccaatactagctataaaagtctggagaagcgggccaggctctcatttgttcccgagacgcctcgcagttcagacgtgactgttgatcccgctcctctgcgaccgctagcttcgatcaactacgcagacaggtaccaaaacaagtgttctcgtcacgtgggcattaatctgattctgtttccctgcagacaatgcgagagaatgaatcagaactcaaatatctgcttcactcacggacagaaagactgtttagagtgctttcccgtgtcagaatctcaacccgtttctgtcgtcaaaaaggcgtatcagaaactgtgctacattcatcatatcatgggaaaggtgccagacgcttgcactgcctgcgatctggtcaatgtggatttggatgactgcatctttgaacaataaatgacttaagccaggtatggctgccgatggttatcttccagattggctcgaggacaaccttagtgaaggaattcgcgagtggtgggctttgaaacctggagcccctcaacccaaggcaaatcaacaacatcaagacaacgctcgaggtcttgtgcttccgggttacaaataccttggacccggcaacggactcgacaagggggagccggtcaacgcagcagacgcggcggccctcgagcacgacaaggcctacgaccagcagctcaaggccggagacaacccgtacctcaagtacaaccacgccgacgccgagttccaggagcggctcaaagaagatacgtcttttgggggcaacctcgggcgagcagtcttccaggccaaaaagaggcttcttgaacctcttggtctggttgaggaagcggctaagacggctcctggaaagaagaggcctgtagagcagtctcctcaggaaccggactcctccgcgggtattggcaaatcgggtgcacagcccgctaaaaagagactcaatttcggtcagactggcgacacagagtcagtcccagaccctcaaccaatcggagaacctcccgcagccccctcaggtgtgggatctcttacaatggcttcaggtggtggcgcaccagtggcagacaataacgaaggtgccgatggagtgggtagttcctcgggaaattggcattgcgattcccaatggctgggggacagagtcatcaccaccagcacccgaacctgggccctgcccacctacaacaatcacctctacaagcaaatctccaacagcacatctggaggatcttcaaatgacaacgcctacttcggctacagcaccccctgggggtattttgacttcaacagattccactgccacttctcaccacgtgactggcagcgactcatcaacaacaactggggattccggcctaagcgactcaacttcaagctcttcaacattcaggtcaaagaggttacggacaacaatggagtcaagaccatcgccaataaccttaccagcacggtccaggtcttcacggactcagactatcagctcccgtacgtgctcgggtcggctcacgagggctgcctcccgccgttcccagcggacgttttcatgattcctcagtacgggtatctgacgcttaatgatggaagccaggccgtgggtcgttcgtccttttactgcctggaatatttcccgtcgcaaatgctaagaacgggtaacaacttccagttcagctacgagtttgagaacgtacctttccatagcagctacgctcacagccaaagcctggaccgactaatgaatccactcatcgaccaatacttgtactatctctctagaactattaacggttctggacagaatcaacaaacgctaaaattcagtgtggccggacccagcaacatggctgtccagggaagaaactacatacctggacccagctaccgacaacaacgtgtctcaaccactgtgactcaaaacaacaacagcgaatttgcttggcctggagcttcttcttgggctctcaatggacgtaatagcttgatgaatcctggacctgctatggccagccacaaagaaggagaggaccgtttctttcctttgtctggatctttaatttttggcaaacaaggtaccggcagagacaacgtggatgcggacaaagtcatgataaccaacgaagaagaaattaaaactactaacccggtagcaacggagtcctatggacaagtggccacaaaccaccagagtgcccaaactttggcggtgccttttaaggcacaggcgcagaccggttgggttcaaaaccaaggaatacttccgggtatggtttggcaggacagagatgtgtacctgcaaggacccatttgggccaaaattcctcacacggacggcaactttcacccttctccgctgatgggagggtttggaatgaagcacccgcctcctcagatcctcatcaaaaacacacctgtacctgcggatcctccaacggccttcaacaaggacaagctgaactctttcatcacccagtattctactggccaagtcagcgtggagatcgagtgggagctgcagaaggaaaacagcaagcgctggaacccggagatccagtacacttccaactattacaagtctaataatgttgaatttgctgttaatactgaaggtgtatatagtgaaccccgccccattggcaccagatacctgactcgtaatctgtaagtcgacttgcttgttaatcaataaaccgtttaattcgtttcagttgaactttggtctctgcgaagggcaattcgtttaaacctgcaggactagaggtcctgtattagaggtcacgtgagtgttttgcgacattttgcgacaccatgtggtcacgctgggtatttaagcccgagtgagcacgcagggtctccattttgaagcgggaggtttgaacgcgcagccgccaagccgaattctgcagatatcacatgtcctaggaactatcgatccatcacactggcggccgctcgactagagcggccgccaccgcggtggagctccagcttttgcggaccgaatcggaaagaacatgtgagcaaaaggccagcaaaaggccaggaaccgtaaaaaggccgcgttgctggcgtttttccataggctccgcccccctgacgagcatcacaaaaatcgacgctcaagtcagaggtggcgaaacccgacaggactataaagataccaggcgtttccccctggaagctccctcgtgcgctctcctgttccgaccctgccgcttaccggatacctgtccgcctttctcccttcgggaagcgtggcgctttctcatagctcacgctgtaggtatctcagttcggtgtaggtcgttcgctccaagctgggctgtgtgcacgaaccccccgttcagcccgaccgctgcgccttatccggtaactatcgtcttgagtccaacccggtaagacacgacttatcgccactggcagcagccactggtaacaggattagcagagcgaggtatgtaggcggtgctacagagttcttgaagtggtggcctaactacggctacactagaagaacagtatttggtatctgcgctctgctgaagccagttaccttcggaaaaagagttggtagctcttgatccggcaaacaaaccaccgctggtagcggtggtttttttgtttgcaagcagcagattacgcgcagaaaaaaaggatctcaagaagatcctttgatcttttctacggggtctgacgctcagtggaacgaaaactcacgttaagggattttggtcatgagattatcaaaaaggatcttcacctagatccttttaaattaaaaatgaagttttaaatcaatctaaagtatatatgagtaaacttggtctgacagttaccaatgcttaatcagtgaggcacctatctcagcgatctgtctatttcgttcatccatagttgcctgactccccgtcgtgtagataactacgatacgggagggcttaccatctggccccagtgctgcaatgataccgcgagacccacgctcaccggctccagatttatcagcaataaaccagccagccggaagggccgagcgcagaagtggtcctgcaactttatccgcctccatccagtctattaattgttgccgggaagctagagtaagtagttcgccagttaatagtttgcgcaacgttgttgccattgctacaggcatcgtggtgtcacgctcgtcgtttggtatggcttcattcagctccggttcccaacgatcaaggcgagttacatgatcccccatgttgtgcaaaaaagcggttagctccttcggtcctccgatcgttgtcagaagtaagttggccgcagtgttatcactcatggttatggcagcactgcataattctcttactgtcatgccatccgtaagatgcttttctgtgactggtgagtactcaaccaagtcattctgagaatagtgtatgcggcgaccgagttgctcttgcccggcgtcaatacgggataataccgcgccacatagcagaactttaaaagtgctcatcattggaaaacgttcttcggggcgaaaactctcaaggatcttaccgctgttgagatccagttcgatgtaacccactcgtgcacccaactgatcttcagcatcttttactttcaccagcgtttctgggtgagcaaaaacaggaaggcaaaatgccgcaaaaaagggaataagggcgacacggaaatgttgaatactcatactcttcctttttcaatattattgaagcatttatcagggttattgtctcatgagcggatacatatttgaatgtatttagaaaaataaacaaataggggttccgcgcacatttccccgaaaagtgccacctgacgtc

SEQ ID NO: 29 - DNA, 11635 bp, synthetic construct
  source 1..11635: mol_type = other DNA
ggtacccaactccatgcttaacagtccccaggtacagcccaccctgcgtcgcaaccaggaacagctctacagcttcctggagcgccactcgccctacttccgcagccacagtgcgcagattaggagcgccacttctttttgtcacttgaaaaacatgtaaaaataatgtactaggagacactttcaataaaggcaaatgtttttatttgtacactctcgggtgattatttaccccccacccttgccgtctgcgccgtttaaaaatcaaaggggttctgccgcgcatcgctatgcgccactggcagggacacgttgcgatactggtgtttagtgctccacttaaactcaggcacaaccatccgcggcagctcggtgaagttttcactccacaggctgcgcaccatcaccaacgcgtttagcaggtcgggcgccgatatcttgaagtcgcagttggggcctccgccctgcgcgcgcgagttgcgatacacagggttgcagcactggaacactatcagcgccgggtggtgcacgctggccagcacgctcttgtcggagatcagatccgcgtccaggtcctccgcgttgctcagggcgaacggagtcaactttggtagctgccttcccaaaaagggtgcatgcccaggctttgagttgcactcgcaccgtagtggcatcagaaggtgaccgtgcccggtctgggcgttaggatacagcgcctgcatgaaagccttgatctgcttaaaagccacctgagcctttgcgccttcagagaagaacatgccgcaagacttgccggaaaactgattggccggacaggccgcgtcatgcacgcagcaccttgcgtcggtgttggagatctgcaccacatttcggccccaccggttcttcacgatcttggccttgctagactgctccttcagcgcgcgctgcccgttttcgctcgtcacatccatttcaatcacgtgctccttatttatcataatgctcccgtgtagacacttaagctcgccttcgatctcagcgcagcggtgcagccacaacgcgcagcccgtgggctcgtggtgcttgtaggttacctctgcaaacgactgcaggtacgcctgcaggaatcgccccatcatcgtcacaaaggtcttgttgctggtgaaggtcagctgcaacccgcggtgctcctcgtttagccaggtcttgcatacggccgccagagcttccacttggtcaggcagtagcttgaagtttgcctttagatcgttatccacgtggtacttgtccatcaacgcgcgcgcagcctccatgcccttctcccacgcagacacgatcggcaggctcagcgggtttatcaccgtgctttcactttccgcttcactggactcttccttttcctcttgcgtccgcataccccgcgccactgggtcgtcttcattcagccgccgcaccgtgcgcttacctcccttgccgtgcttgattagcaccggtgggttgctgaaacccaccatttgtagcgccacatcttctctttcttcctcgctgtccacgatcacctctggggatggcgggcgctcgggcttgggagaggggcgcttctttttctttttggacgcaatggccaaatccgccgtcgaggtcgatggccgcgggctgggtgtgcgcggcaccagcgcatcttgtgacgagtcttcttcgtcctcggactcgagacgccgcctcagccgcttttttgggggcgcgcggggaggcggcggcgacggcgacggggacgacacgtcctccatggttggtggacgtcgcgccgcaccgcgtccgcgctcgggggtggtttcgcgctgctcctcttcccgactggccatttccttctcctataggcagaaaaagatcatggagtcagtcgagaaggaggacagcctaaccgccccctttgagttcgccaccaccgcctccaccgatgccgccaacgcgcctaccaccttccccgtcgaggcacccccgcttgaggaggaggaagtgattatcgagcaggacccaggttttgtaagcgaagacgacgaggatcgctcagtaccaacagaggataaaaagcaagaccaggacgacgcagaggcaaacgaggaacaagtcgggcggggggaccaaaggcatggcgactacctagatgtgggagacgacgtgctgttgaagcatctgcagcgccagtgcgccattatctgcgacgcgttgcaagagcgcagcgatgtgcccctcgccatagcggatgtcagccttgcctacgaacgccacctgttctcaccgcgcgtaccccccaaacgccaagaaaacggcacatgcgagcccaacccgcgcctcaacttctaccccgtatttgccgtgccagaggtgcttgccacctatcacatctttttccaaaactgcaagatacccctatcctgccgtgccaaccgcagccgagcggacaagcagctggccttgcggcagggcgctgtcatacctgatatcgcctcgctcgacgaagtgccaaaaatctttgagggtcttggacgcgacgagaaacgcgcggcaaacgctctgcaacaagaaaacagcgaaaatgaaagtcactgtggagtgctggtggaacttgagggtgacaacgcgcgcctagccgtgctgaaacgcagcatcgaggtcacccactttgcctacccggcacttaacctaccccccaaggttatgagcacagtcatgagcgagctgatcgtgcgccgtgcacgacccctggagagggatgcaaacttgcaagaacaaaccgaggagggcctacccgcagttggcgatgagcagctggcgcgctggcttgagacgcgcgagcctgccgacttggaggagcgacgcaagctaatgatggccgcagtgcttgttaccgtggagcttgagtgcatgcagcggttctttgctgacccggagatgcagcgcaagctagaggaaacgttgcactacacctttcgccagggctacgtgcgccaggcctgcaaaatttccaacgtggagctctgcaacctggtctcctaccttggaattttgcacgaaaaccgcctcgggcaaaacgtgcttcattccacgctcaagggcgaggcgcgccgcgactacgtccgcgactgcgtttacttatttctgtgctacacctggcaaacggccatgggcgtgtggcagcaatgcctggaggagcgcaacctaaaggagctgcagaagctgctaaagcaaaacttgaaggacctatggacggccttcaacgagcgctccgtggccgcgcacctggcggacattatcttccccgaacgcctgcttaaaaccctgcaacagggtctgccagacttcaccagtcaaagcatgttgcaaaactttaggaactttatcctagagcgttcaggaattctgcccgccacctgctgtgcgcttcctagcgactttgtgcccattaagtaccgtgaatgccctccgccgctttggggtcactgctaccttctgcagctagccaactaccttgcctaccactccgacatcatggaagacgtgagcggtgacggcctactggagtgtcactgtcgctgcaacctatgcaccccgcaccgctccctggtctgcaattcgcaactgcttagcgaaagtcaaattatcggtacctttgagctgcagggtccctcgcctgacgaaaagtccgcggctccggggttgaaactcactccggggctgtggacgtcggcttaccttcgcaaatttgtacctgaggactaccacgcccacgagattaggttctacgaagaccaatcccgcccgccaaatgcggagcttaccgcctgcgtcattacccagggccacatccttggccaattgcaagccatcaacaaagcccgccaagagtttctgctacgaaagggacggggggtttacctggacccccagtccggcgaggagctcaacccaatccccccgccgccgcagccctatcagcagccgcgggcccttgcttcccaggatggcacccaaaaagaagctgcagctgccgccgccgccacccacggacgaggaggaatactgggacagtcaggcagaggaggttttggacgaggaggaggagatgatggaagactgggacagcctagacgaagcttccgaggccgaagaggtgtcagacgaaacaccgtcaccctcggtcgcattcccctcgccggcgccccagaaattggcaaccgttcccagcatcgctacaacctccgctcctcaggcgccgccggcactgcctgttcgccgacccaaccgtagatgggacaccactggaaccagggccggtaagtctaagcagccgccgccgttagcccaagagcaacaacagcgccaaggctaccgctcgtggcgcgggcacaagaacgccatagttgcttgcttgcaagactgtgggggcaacatctccttcgcccgccgctttcttctctaccatcacggcgtggccttcccccgtaacatcctgcattactaccgtcatctctacagcccctactgcaccggcggcagcggcagcggcagcaacagcagcggtcacacagaagcaaaggcgaccggatagcaagactctgacaaagcccaagaaatccacagcggcggcagcagcaggaggaggagcgctgcgtctggcgcccaacgaacccgtatcgacccgcgagcttagaaataggatttttcccactctgtatgctatatttcaacaaagcaggggccaagaacaagagctgaaaataaaaaacaggtctctgcgctccctcacccgcagctgcctgtatcacaaaagcgaagatcagcttcggcgcacgctggaagacgcggaggctctcttcagcaaatactgcgcgctgactcttaaggactagtttcgcgccctttctcaaatttaagcgcgaaaactacgtcatctccagcggccacacccggcgccagcacctgtcgtcagcgccattatgagcaaggaaattcccacgccctacatgtggagttaccagccacaaatgggacttgcggctggagctgcccaagactactcaacccgaataaactacatgagcgcgggaccccacatgatatcccgggtcaacggaatccgcgcccaccgaaaccgaattctcctcgaacaggcggctattaccaccacacctcgtaataaccttaatccccgtagttggcccgctgccctggtgtaccaggaaagtcccgctcccaccactgtggtacttcccagagacgcccaggccgaagttcagatgactaactcaggggcgcagcttgcgggcggctttcgtcacagggtgcggtcgcccgggcgttttagggcggagtaacttgcatgtattgggaattgtagtttttttaaaatgggaagtgacgtatcgtgggaaaacggaagtgaagatttgaggaagttgtgggttttttggctttcgtttctgggcgtaggttcgcgtgcggttttctgggtgttttttgtggactttaaccgttacgtcattttttagtcctatatatactcgctctgtacttggccctttttacactgtgactgattgagctggtgccgtgtcgagtggtgttttttaataggtttttttactggtaaggctgactgttatggctgccgctgtggaagcgctgtatgttgttctggagcgggagggtgctattttgcctaggcaggagggtttttcaggtgtttatgtgtttttctctcctattaattttgttatacctcctatgggggctgtaatgttgtctctacgcctgcgggtatgtattcccccgggctatttcggtcgctttttagcactgaccgatgttaaccaacctgatgtgtttaccgagtcttacattatgactccggacatgaccgaggaactgtcggtggtgctttttaatcacggtgaccagtttttttacggtcacgccggcatggccgtagtccgtcttatgcttataagggttgtttttcctgttgtaagacaggcttctaatgtttaaatgtttttttttttgttattttattttgtgtttaatgcaggaacccgcagacatgtttgagagaaaaatggtgtctttttctgtggtggttccggaacttacctgcctttatctgcatgagcatgactacgatgtgcttgcttttttgcgcgaggctttgcctgattttttgagcagcaccttgcattttatatcgccgcccatgcaacaagcttacataggggctacgctggttagcatagctccgagtatgcgtgtcataatcagtgtgggttcttttgtcatggttcctggcggggaagtggccgcgctggtccgtgcagacctgcacgattatgttcagctggccctgcgaagggacctacgggatcgcggtatttttgttaatgttccgcttttgaatcttatacaggtctgtgaggaacctgaatttttgcaatcatgattcgctgcttgaggctgaaggtggagggcgctctggagcagatttttacaatggccggacttaatattcgggatttgcttagagacatattgataaggtggcgagatgaaaattatttgggcatggttgaaggtgctggaatgtttatagaggagattcaccctgaagggtttagcctttacgtccacttggacgtgagggcagtttgccttttggaagccattgtgcaacatcttacaaatgccattatctgttctttggctgtagagtttgaccacgccaccggaggggagcgcgttcacttaatagatcttcattttgaggttttggataatcttttggaataaaaaaaaaaaaacatggttcttccagctcttcccgctcctcccgtgtgtgactcgcagaacgaatgtgtaggttggctgggtgtggcttattctgcggtggtggatgttatcagggcagcggcgcatgaaggagtttacatagaacccgaagccagggggcgcctggatgctttgagagagtggatatactacaactactacacagagcgagctaagcgacgagaccggagacgcagatctgtttgtcacgcccgcacctggttttgcttcaggaaatatgactacgtccggcgttccatttggcatgacactacgaccaacacgatctcggttgtctcggcgcactccgtacagtagggatcgcctacctccttttgagacagagacccgcgctaccatactggaggatcatccgctgctgcccgaatgtaacactttgacaatgcacaacgtgagttacgtgcgaggtcttccctgcagtgtgggatttacgctgattcaggaatgggttgttccctgggatatggttctgacgcgggaggagcttgtaatcctgaggaagtgtatgcacgtgtgcctgtgttgtgccaacattgatatcatgacgagcatgatgatccatggttacgagtcctgggctctccactgtcattgttccagtcccggttccctgcagtgcatagccggcgggcaggttttggccagctggtttaggatggtggtggatggcgccatgtttaatcagaggtttatatggtaccgggaggtggtgaattacaacatgccaaaagaggtaatgtttatgtccagcgtgtttatgaggggtcgccacttaatctacctgcgcttgtggtatgatggccacgtgggttctgtggtccccgccatgagctttggatacagcgccttgcactgtgggattttgaacaatattgtggtgctgtgctgcagttactgtgctgatttaagtgagatcagggtgcgctgctgtgcccggaggacaaggcgtctcatgctgcgggcggtgcgaatcatcgctgaggagaccactgccatgttgtattcctgcaggacggagcggcggcggcagcagtttattcgcgcgctgctgcagcaccaccgccctatcctgatgcacgattatgactctacccccatgtaggcgtggacttccccttcgccgcccgttgagcaaccgcaagttggacagcagcctgtggctcagcagctggacagcgacatgaacttaagcgagctgcccggggagtttattaatatcactgatgagcgtttggctcgacaggaaaccgtgtggaatataacacctaagaatatgtctgttacccatgatatgatgctttttaaggccagccggggagaaaggactgtgtactctgtgtgttgggagggaggtggcaggttgaatactagggttctgtgagtttgattaaggtacggtgatcaatataagctatgtggtggtggggctatactactgaatgaaaaatgacttgaaattttctgcaattgaaaaataaacacgttgaaacataacatgcaacaggttcacgattctttattcctgggcaatgtaggagaaggtgtaagagttggtagcaaaagtttcagtggtgtattttccactttcccaggaccatgtaaaagacatagagtaagtgcttacctcgctagtttctgtggattcactagaatcgatgtaggatgttgcccctcctgacgcggtaggagaaggggagggtgccctgcatgtctgccgctgctcttgctcttgccgctgctgaggaggggggcgcatctgccgcagcaccggatgcatctgggaaaagcaaaaaaggggctcgtccctgtttccggaggaatttgcaagcggggtcttgcatgacggggaggcaaacccccgttcgccgcagtccggccggcccgagactcgaaccgggggtcctgcgactcaacccttggaaaataaccctccggctacagggagcgagccacttaatgctttcgctttccagcctaaccgcttacgccgcgcgcggccagtggccaaaaaagctagcgcagcagccgccgcgcctggaaggaagccaaaaggagcgctcccccgttgtctgacgtcgcacacctgggttcgacacgcgggcggtaaccgcatggatcacggcggacggccggatccggggttcgaaccccggtcgtccgccatgatacccttgcgaatttatccaccagaccacggaagagtgcccgcttacaggctctccttttgcacggtctagagcgtcaacgactgcgcacgcctcaccggccagagcgtcccgaccatggagcactttttgccgctgcgcaacatctggaaccgcgtccgcgactttccgcgcgcctccaccaccgccgccggcatcacctggatgtccaggtacatctacggattacgtcgacgtttaaaccatatgatcagctcactcaaaggcggtaatacggttatccacagaatcaggggataacgcaggaaagaacatgtgagcaaaaggccagcaaaaggccaggaaccgtaaaaaggccgcgttgctggcgtttttccataggctccgcccccctgacgagcatcacaaaaatcgacgctcaagtcagaggtggcgaaacccgacaggactataaagataccaggcgtttccccctggaagctccctcgtgcgctctcctgttccgaccctgccgcttaccggatacctgtccgcctttctcccttcgggaagcgtggcgctttctcatagctcacgctgtaggtatctcagttcggtgtaggtcgttcgctccaagctgggctgtgtgcacgaaccccccgttcagcccgaccgctgcgccttatccggtaactatcgtcttgagtccaacccggtaagacacgacttatcgccactggcagcagccactggtaacaggattagcagagcgaggtatgtaggcggtgctacagagttcttgaagtggtggcctaactacggctacactagaagaacagtatttggtatctgcgctctgctgaagccagttaccttcggaaaaagagttggtagctcttgatccggcaaacaaaccaccgctggtagcggtggtttttttgtttgcaagcagcagattacgcgcagaaaaaaaggatctcaagaagatcctttgatcttttctacggggtctgacgctcagtggaacgaaaactcacgttaagggattttggtcatgagattatcaaaaaggatcttcacctagatccttttaaattaaaaatgaagttttaaatcaatctaaagtatatatgagtaaacttggtctgacagttaccaatgcttaatcagtgaggcacctatctcagcgatctgtctatttcgttcatccatagttgcctgactccccgtcgtgtagataactacgatacgggagggcttaccatctggccccagtgctgcaatgataccgcgagacccacgctcaccggctccagatttatcagcaataaaccagccagccggaagggccgagcgcagaagtggtcctgcaactttatccgcctccatccagtctattaattgttgccgggaagctagagtaagtagttcgccagttaatagtttgcgcaacgttgttgccattgctacaggcatcgtggtgtcacgctcgtcgtttggtatggcttcattcagctccggttcccaacgatcaaggcgagttacatgatcccccatgttgtgcaaaaaagcggttagctccttcggtcctccgatcgttgtcagaagtaagttggccgcagtgttatcactcatggttatggcagcactgcataattctcttactgtcatgccatccgtaagatgcttttctgtgactggtgagtactcaaccaagtcattctgagaatagtgtatgcggcgaccgagttgctcttgcccggcgtcaatacgggataataccgcgccacatagcagaactttaaaagtgctcatcattggaaaacgttcttcggggcgaaaactctcaaggatcttaccgctgttgagatccagttcgatgtaacccactcgtgcacccaactgatcttcagcatcttttactttcaccagcgtttctgggtgagcaaaaacaggaaggcaaaatgccgcaaaaaagggaataagggcgacacggaaatgttgaatactcatactcttcctttttcaatattattgaagcatttatcagggttattgtctcatgagcggatacatatttgaatgtatttagaaaaataaacaaataggggttccgcgcacatttccccgaaaagtgccacctaaattgtaagcgttaatattttgttaaaattcgcgttaaatttttgttaaatcagctcattttttaaccaataggccgaaatcggcaaaatcccttataaatcaaaagaatagaccgagatagggttgagtgttgttccagtttggaacaagagtccactattaaagaacgtggactccaacgtcaaagggcgaaaaaccgtctatcagggcgatggcccactacgtgaaccatcaccctaatcaagttttttggggtcgaggtgccgtaaagcactaaatcggaaccctaaagggagcccccgatttagagcttgacggggaaagccggcgaacgtggcgagaaaggaagggaagaaagcgaaaggagcgggcgctagggcgctggcaagtgtagcggtcacgctgcgcgtaaccaccacacccgccgcgcttaatgcgccgctacagggcgcgatggatcc

SEQ ID NO: 30 - DNA, 25 bp, synthetic construct
  source 1..25: mol_type = other DNA
actttccattgacgtcaatgggtgg

SEQ ID NO: 31 - DNA, 29 bp, synthetic construct
  source 1..29: mol_type = other DNA
caagtgtatcatatgccaagtacgccccc

SEQ ID NO: 32 - DNA, 23 bp, synthetic construct
  source 1..23: mol_type = other DNA
aggtcatgtactgggcataatgc

SEQ ID NO: 33 - protein, 724 aa, Adeno-associated virus 5
MSFVDHPPDWLEEVGEGLREFLGLEAGPPKPKPNQQHQDQARGLVLPGYNYLGPGNGLDRGEPVNRADEVAREHDISYNEQLEAGDNPYLKYNHADAEFQEKLADDTSFGGNLGKAVFQAKKRVLEPFGLVEEGAKTAPTGKRIDDHFPKRKKARTEEDSKPSTSSDAEAGPSGSQQLQIPAQPASSLGADTMSAGGGGPLGDNNQGADGVGNASGDWHCDSTWMGDRVVTKSTRTWVLPSYNNHQYREIKSGSVDGSNANAYFGYSTPWGYFDFNRFHSHWSPRDWQRLINNYWGFRPRSLRVKIFNIQVKEVTVQDSTTTIANNLTSTVQVFTDDDYQLPYVVGNGTEGCLPAFPPQVFTLPQYGYATLNRDNTENPTERSSFFCLEYFPSKMLRTGNNFEFTYNFEEVPFHSSFAPSQNLFKLANPLVDQYLYRFVSTNNTGGVQFNKNLAGRYANTYKNWFPGPMGRTQGWNLGSGVNRASVSAFATTNRMELEGASYQVPPQPNGMTNNLQGSNTYALENTMIFNSQPANPGTTATYLEGNMLITSESETQPVNRVAYNVGGQMATNNQSSTTAPATGTYNLQEIVPGSVWMERDVYLQGPIWAKIPETGAHFHPSPAMGGFGLKHPPPMMLIKNTPVPGNITSFSDVPVSSFITQYSTGQVTVEMEWELKKENSKRWNPEIQYTNNYNDPQFVDFAPDSTGEYRTTRPIGTRYLTRPL

SEQ ID NO: 34 - protein, 736 aa, Adeno-associated virus 9
MAADGYLPDWLEDNLSEGIREWWALKPGAPQPKANQQHQDNARGLVLPGYKYLGPGNGLDKGEPVNAADAAALEHDKAYDQQLKAGDNPYLKYNHADAEFQERLKEDTSFGGNLGRAVFQAKKRLLEPLGLVEEAAKTAPGKKRPVEQSPQEPDSSAGIGKSGAQPAKKRLNFGQTGDTESVPDPQPIGEPPAAPSGVGSLTMASGGGAPVADNNEGADGVGSSSGNWHCDSQWLGDRVITTSTRTWALPTYNNHLYKQISNSTSGGSSNDNAYFGYSTPWGYFDFNRFHCHFSPRDWQRLINNNWGFRPKRLNFKLFNIQVKEVTDNNGVKTIANNLTSTVQVFTDSDYQLPYVLGSAHEGCLPPFPADVFMIPQYGYLTLNDGSQAVGRSSFYCLEYFPSQMLRTGNNFQFSYEFENVPFHSSYAHSQSLDRLMNPLIDQYLYYLSKTINGSGQNQQTLKFSVAGPSNMAVQGRNYIPGPSYRQQRVSTTVTQNNNSEFAWPGASSWALNGRNSLMNPGPAMASHKEGEDRFFPLSGSLIFGKQGTGRDNVDADKVMITNEEEIKTTNPVATESYGQVATNHQSAQAQAQTGWVQNQGILPGMVWQDRDVYLQGPIWAKIPHTDGNFHPSPLMGGFGMKHPPPQILIKNTPVPADPPTAFNKDKLNSFITQYSTGQVSVEIEWELQKENSKRWNPEIQYTSNYYKSNNVEFAVNTEGVYSEPRPIGTRYLTRNL

SEQ ID NO: 35 - protein, 743 aa, synthetic construct
MAADGYLPDWLEDNLSEGIREWWALKPGAPQPKANQQHQDNARGLVLPGYKYLGPGNGLDKGEPVNAADAAALEHDKAYDQQLKAGDNPYLKYNHADAEFQERLKEDTSFGGNLGRAVFQAKKRLLEPLGLVEEAAKTAPGKKRPVEQSPQEPDSSAGIGKSGAQPAKKRLNFGQTGDTESVPDPQPIGEPPAAPSGVGSLTMASGGGAPVADNNEGADGVGSSSGNWHCDSQWLGDRVITTSTRTWALPTYNNHLYKQISNSTSGGSSNDNAYFGYSTPWGYFDFNRFHCHFSPRDWQRLINNNWGFRPKRLNFKLFNIQVKEVTDNNGVKTIANNLTSTVQVFTDSDYQLPYVLGSAHEGCLPPFPADVFMIPQYGYLTLNDGSQAVGRSSFYCLEYFPSQMLRTGNNFQFSYEFENVPFHSSYAHSQSLDRLMNPLIDQYLYYLSRTINGSGQNQQTLKFSVAGPSNMAVQGRNYIPGPSYRQQRVSTTVTQNNNSEFAWPGASSWALNGRNSLMNPGPAMASHKEGEDRFFPLSGSLIFGKQGTGRDNVDADKVMITNEEEIKTTNPVATESYGQVATNHQSDGTLAVPFKAQAQTGWVQNQGILPGMVWQDRDVYLQGPIWAKIPHTDGNFHPSPLMGGFGMKHPPPQILIKNTPVPADPPTAFNKDKLNSFITQYSTGQVSVEIEWELQKENSKRWNPEIQYTSNYYKSNNVEFAVNTEGVYSEPRPIGTRYLTRNL

SEQ ID NO: 36 - protein, 743 aa, synthetic construct
MAADGYLPDWLEDNLSEGIREWWALKPGAPQPKANQQHQDNARGLVLPGYKYLGPGNGLDKGEPVNAADAAALEHDKAYDQQLKAGDNPYLKYNHADAEFQERLKEDTSFGGNLGRAVFQAKKRLLEPLGLVEEAAKTAPGKKRPVEQSPQEPDSSAGIGKSGAQPAKKRLNFGQTGDTESVPDPQPIGEPPAAPSGVGSLTMASGGGAPVADNNEGADGVGSSSGNWHCDSQWLGDRVITTSTRTWALPTYNNHLYKQISNSTSGGSSNDNAYFGYSTPWGYFDFNRFHCHFSPRDWQRLINNNWGFRPKRLNFKLFNIQVKEVTDNNGVKTIANNLTSTVQVFTDSDYQLPYVLGSAHEGCLPPFPADVFMIPQYGYLTLNDGSQAVGRSSFYCLEYFPSQMLRTGNNFQFSYEFENVPFHSSYAHSQSLDRLMNPLIDQYLYYLSRTINGSGQNQQTLKFSVAGPSNMAVQGRNYIPGPSYRQQRVSTTVTQNNNSEFAWPGASSWALNGRNSLMNPGPAMASHKEGEDRFFPLSGSLIFGKQGTGRDNVDADKVMITNEEEIKTTNPVATESYGQVATNHQSAQQAVRTSLAQAQTGWVQNQGILPGMVWQDRDVYLQGPIWAKIPHTDGNFHPSPLMGGFGMKHPPPQILIKNTPVPADPPTAFNKDKLNSFITQYSTGQVSVEIEWELQKENSKRWNPEIQYTSNYYKSNNVEFAVNTEGVYSEPRPIGTRYLTRNL

SEQ ID NO: 37 - protein, 743 aa, synthetic construct
MAADGYLPDWLEDNLSEGIREWWALKPGAPQPKANQQHQDNARGLVLPGYKYLGPGNGLDKGEPVNAADAAALEHDKAYDQQLKAGDNPYLKYNHADAEFQERLKEDTSFGGNLGRAVFQAKKRLLEPLGLVEEAAKTAPGKKRPVEQSPQEPDSSAGIGKSGAQPAKKRLNFGQTGDTESVPDPQPIGEPPAAPSGVGSLTMASGGGAPVADNNEGADGVGSSSGNWHCDSQWLGDRVITTSTRTWALPTYNNHLYKQISNSTSGGSSNDNAYFGYSTPWGYFDFNRFHCHFSPRDWQRLINNNWGFRPKRLNFKLFNIQVKEVTDNNGVKTIANNLTSTVQVFTDSDYQLPYVLGSAHEGCLPPFPADVFMIPQYGYLTLNDGSQAVGRSSFYCLEYFPSQMLRTGNNFQFSYEFENVPFHSSYAHSQSLDRLMNPLIDQYLYYLSRTINGSGQNQQTLKFSVAGPSNMAVQGRNYIPGPSYRQQRVSTTVTQNNNSEFAWPGASSWALNGRNSLMNPGPAMASHKEGEDRFFPLSGSLIFGKQGTGRDNVDADKVMITNEEEIKTTNPVATESYGQVATNHQSAQTLAVPFKAQAQTGWVQNQGILPGMVWQDRDVYLQGPIWAKIPHTDGNFHPSPLMGGFGMKHPPPQILIKNTPVPADPPTAFNKDKLNSFITQYSTGQVSVEIEWELQKENSKRWNPEIQYTSNYYKSNNVEFAVNTEGVYSEPRPIGTRYLTRNL

SEQ ID NO: 38 - DNA, 2175 bp, Adeno-associated virus 5
  source 1..2175: mol_type = genomic DNA
atgtcttttgttgatcaccctccagattggttggaagaagttggtgaaggtcttcgcgagtttttgggccttgaagcgggcccaccgaaaccaaaacccaatcagcagcatcaagatcaagcccgtggtcttgtgctgcctggttataactatctcggacccggaaacggtctcgatcgaggagagcctgtcaacagggcagacgaggtcgcgcgagagcacgacatctcgtacaacgagcagcttgaggcgggagacaacccctacctcaagtacaaccacgcggacgccgagtttcaggagaagctcgccgacgacacatccttcgggggaaacctcggaaaggcagtctttcaggccaagaaaagggttctcgaaccttttggcctggttgaagagggtgctaagacggcccctaccggaaagcggatagacgaccactttccaaaaagaaagaaggctcggaccgaagaggactccaagccttccacctcgtcagacgccgaagctggacccagcggatcccagcagctgcaaatcccagcccaaccagcctcaagtttgggagctgatacaatgtctgcgggaggtggcggcccattgggcgacaataaccaaggtgccgatggagtgggcaatgcctcgggagattggcattgcgattccacgtggatgggggacagagtcgtcaccaagtccacccgaacctgggtgctgcccagctacaacaaccaccagtaccgagagatcaaaagcggctccgtcgacggaagcaacgccaacgcctactttggatacagcaccccctgggggtactttgactttaaccgcttccacagccactggagcccccgagactggcaaagactcatcaacaactactggggcttcagaccccggtccctcagagtcaaaatcttcaacattcaagtcaaagaggtcacggtgcaggactccaccaccaccatcgccaacaacctcacctccaccgtccaagtgtttacggacgacgactaccagctgccctacgtcgtcggcaacgggaccgagggatgcctgccggccttccctccgcaggtctttacgctgccgcagtacggttacgcgacgctgaaccgcgacaacacagaaaatcccaccgagaggagcagcttcttctgcctagagtactttcccagcaagatgctgagaacgggcaacaactttgagtttacctacaactttgaggaggtgcccttccactccagcttcgctcccagtcagaacctgttcaagctggccaacccgctggtggaccagtacttgtaccgcttcgtgagcacaaataacactggcggagtccagttcaacaagaacctggccgggagatacgccaacacctacaaaaactggttcccggggcccatgggccgaacccagggctggaacctgggctccggggtcaaccgcgccagtgtcagcgccttcgccacgaccaataggatggagctcgagggcgcgagttaccaggtgcccccgcagccgaacggcatgaccaacaacctccagggcagcaacacctatgccctggagaacactatgatcttcaacagccagccggcgaacccgggcaccaccgccacgtacctcgagggcaacatgctcatcaccagcgagagcgagacgcagccggtgaaccgcgtggcgtacaacgtcggcgggcagatggccaccaacaaccagagctccaccactgcccccgcgaccggcacgtacaacctccaggaaatcgtgcccggcagcgtgtggatggagagggacgtgtacctccaaggacccatctgggccaagatcccagagacgggggcgcactttcacccctctccggccatgggcggattcggactcaaacacccaccgcccatgatgctcatcaagaacacgcctgtgcccggaaatatcaccagcttctcggacgtgcccgtcagcagcttcatcacccagtacagcaccgggcaggtcaccgtggagatggagtgggagctcaagaaggaaaactccaagaggtggaacccagagatccagtacacaaacaactacaacgacccccagtttgtggactttgccccggacagcaccggggaatacagaaccaccagacctatcggaacccgataccttacccgacccctttaa

SEQ ID NO: 39 - DNA, 2211 bp, Adeno-associated virus 9
  source 1..2211: mol_type = genomic DNA
atggctgccgatggttatcttccagattggctcgaggacaaccttagtgaaggaattcgcgagtggtgggctttgaaacctggagcccctcaacccaaggcaaatcaacaacatcaagacaacgctcgaggtcttgtgcttccgggttacaaataccttggacccggcaacggactcgacaagggggagccggtcaacgcagcagacgcggcggccctcgagcacgacaaggcctacgaccagcagctcaaggccggagacaacccgtacctcaagtacaaccacgccgacgccgagttccaggagcggctcaaagaagatacgtcttttgggggcaacctcgggcgagcagtcttccaggccaaaaagaggcttcttgaacctcttggtctggttgaggaagcggctaagacggctcctggaaagaagaggcctgtagagcagtctcctcaggaaccggactcctccgcgggtattggcaaatcgggtgcacagcccgctaaaaagagactcaatttcggtcagactggcgacacagagtcagtcccagaccctcaaccaatcggagaacctcccgcagccccctcaggtgtgggatctcttacaatggcttcaggtggtggcgcaccagtggcagacaataacgaaggtgccgatggagtgggtagttcctcgggaaattggcattgcgattcccaatggctgggggacagagtcatcaccaccagcacccgaacctgggccctgcccacctacaacaatcacctctacaagcaaatctccaacagcacatctggaggatcttcaaatgacaacgcctacttcggctacagcaccccctgggggtattttgacttcaacagattccactgccacttctcaccacgtgactggcagcgactcatcaacaacaactggggattccggcctaagcgactcaacttcaagctcttcaacattcaggtcaaagaggttacggacaacaatggagtcaagaccatcgccaataaccttaccagcacggtccaggtcttcacggactcagactatcagctcccgtacgtgctcgggtcggctcacgagggctgcctcccgccgttcccagcggacgttttcatgattcctcagtacgggtatctgacgcttaatgatggaagccaggccgtgggtcgttcgtccttttactgcctggaatatttcccgtcgcaaatgctaagaacgggtaacaacttccagttcagctacgagtttgagaacgtacctttccatagcagctacgctcacagccaaagcctggaccgactaatgaatccactcatcgaccaatacttgtactatctctcaaagactattaacggttctggacagaatcaacaaacgctaaaattcagtgtggccggacccagcaacatggctgtccagggaagaaactacatacctggacccagctaccgacaacaacgtgtctcaaccactgtgactcaaaacaacaacagcgaatttgcttggcctggagcttcttcttgggctctcaatggacgtaatagcttgatgaatcctggacctgctatggccagccacaaagaaggagaggaccgtttctttcctttgtctggatctttaatttttggcaaacaaggaactggaagagacaacgtggatgcggacaaagtcatgataaccaacgaagaagaaattaaaactactaacccggtagcaacggagtcctatggacaagtggccacaaaccaccagagtgcccaagcacaggcgcagaccggctgggttcaaaaccaaggaatacttccgggtatggtttggcaggacagagatgtgtacctgcaaggacccatttgggccaaaattcctcacacggacggcaactttcacccttctccgctgatgggagggtttggaatgaagcacccgcctcctcagatcctcatcaaaaacacacctgtacctgcggatcctccaacggccttcaacaaggacaagctgaactctttcatcacccagtattctactggccaagtcagcgtggagatcgagtgggagctgcagaaggaaaacagcaagcgctggaacccggagatccagtacacttccaactattacaagtctaataatgttgaatttgctgttaatactgaaggtgtatatagtgaaccccgccccattggcaccagatacctgactcgtaatctgtaa

SEQ ID NO: 40 - DNA, 2232 bp, synthetic construct
  source 1..2232: mol_type = other DNA
atggctgccgatggttatcttccagattggctcgaggacaaccttagtgaaggaattcgcgagtggtgggctttgaaacctggagcccctcaacccaaggcaaatcaacaacatcaagacaacgctcgaggtcttgtgcttccgggttacaaataccttggacccggcaacggactcgacaagggggagccggtcaacgcagcagacgcggcggccctcgagcacgacaaggcctacgaccagcagctcaaggccggagacaacccgtacctcaagtacaaccacgccgacgccgagttccaggagcggctcaaagaagatacgtcttttgggggcaacctcgggcgagcagtcttccaggccaaaaagaggcttcttgaacctcttggtctggttgaggaagcggctaagacggctcctggaaagaagaggcctgtagagcagtctcctcaggaaccggactcctccgcgggtattggcaaatcgggtgcacagcccgctaaaaagagactcaatttcggtcagactggcgacacagagtcagtcccagaccctcaaccaatcggagaacctcccgcagccccctcaggtgtgggatctcttacaatggcttcaggtggtggcgcaccagtggcagacaataacgaaggtgccgatggagtgggtagttcctcgggaaattggcattgcgattcccaatggctgggggacagagtcatcaccaccagcacccgaacctgggccctgcccacctacaacaatcacctctacaagcaaatctccaacagcacatctggaggatcttcaaatgacaacgcctacttcggctacagcaccccctgggggtattttgacttcaacagattccactgccacttctcaccacgtgactggcagcgactcatcaacaacaactggggattccggcctaagcgactcaacttcaagctcttcaacattcaggtcaaagaggttacggacaacaatggagtcaagaccatcgccaataaccttaccagcacggtccaggtcttcacggactcagactatcagctcccgtacgtgctcgggtcggctcacgagggctgcctcccgccgttcccagcggacgttttcatgattcctcagtacgggtatctgacgcttaatgatggaagccaggccgtgggtcgttcgtccttttactgcctggaatatttcccgtcgcaaatgctaagaacgggtaacaacttccagttcagctacgagtttgagaacgtacctttccatagcagctacgctcacagccaaagcctggaccgactaatgaatccactcatcgaccaatacttgtactatctctctagaactattaacggttctggacagaatcaacaaacgctaaaattcagtgtggccggacccagcaacatggctgtccagggaagaaactacatacctggacccagctaccgacaacaacgtgtctcaaccactgtgactcaaaacaacaacagcgaatttgcttggcctggagcttcttcttgggctctcaatggacgtaatagcttgatgaatcctggacctgctatggccagccacaaagaaggagaggaccgtttctttcctttgtctggatctttaatttttggcaaacaaggtaccggcagagacaacgtggatgcggacaaagtcatgataaccaacgaagaagaaattaaaactactaacccggtagcaacggagtcctatggacaagtggccacaaaccaccagagtgatgggactttggcggtgccttttaaggcacaggcgcagaccggttgggttcaaaaccaaggaatacttccgggtatggtttggcaggacagagatgtgtacctgcaaggacccatttgggccaaaattcctcacacggacggcaactttcacccttctccgctgatgggagggtttggaatgaagcacccgcctcctcagatcctcatcaaaaacacacctgtacctgcggatcctccaacggccttcaacaaggacaagctgaactctttcatcacccagtattctactggccaagtcagcgtggagatcgagtgggagctgcagaaggaaaacagcaagcgctggaacccggagatccagtacacttccaactattacaagtctaataatgttgaatttgctgttaatactgaaggtgtatatagtgaaccccgccccattggcaccagatacctgactcgtaatctgtaa

SEQ ID NO: 41 - DNA, 2232 bp, synthetic construct
  source 1..2232: mol_type = other DNA
atggctgccgatggttatcttccagattggctcgaggacaaccttagtgaaggaattcgcgagtggtgggctttgaaacctggagcccctcaacccaaggcaaatcaacaacatcaagacaacgctcgaggtcttgtgcttccgggttacaaataccttggacccggcaacggactcgacaagggggagccggtcaacgcagcagacgcggcggccctcgagcacgacaaggcctacgaccagcagctcaaggccggagacaacccgtacctcaagtacaaccacgccgacgccgagttccaggagcggctcaaagaagatacgtcttttgggggcaacctcgggcgagcagtcttccaggccaaaaagaggcttcttgaacctcttggtctggttgaggaagcggctaagacggctcctggaaagaagaggcctgtagagcagtctcctcaggaaccggactcctccgcgggtattggcaaatcgggtgcacagcccgctaaaaagagactcaatttcggtcagactggcgacacagagtcagtcccagaccctcaaccaatcggagaacctcccgcagccccctcaggtgtgggatctcttacaatggcttcaggtggtggcgcaccagtggcagacaataacgaaggtgccgatggagtgggtagttcctcgggaaattggcattgcgattcccaatggctgggggacagagtcatcaccaccagcacccgaacctgggccctgcccacctacaacaatcacctctacaagcaaatctccaacagcacatctggaggatcttcaaatgacaacgcctacttcggctacagcaccccctgggggtattttgacttcaacagattccactgccacttctcaccacgtgactggcagcgactcatcaacaacaactggggattccggcctaagcgactcaacttcaagctcttcaacattcaggtcaaagaggttacggacaacaatggagtcaagaccatcgccaataaccttaccagcacggtccaggtcttcacggactcagactatcagctcccgtacgtgctcgggtcggctcacgagggctgcctcccgccgttcccagcggacgttttcatgattcctcagtacgggtatctgacgcttaatgatggaagccaggccgtgggtcgttcgtccttttactgcctggaatatttcccgtcgcaaatgctaagaacgggtaacaacttccagttcagctacgagtttgagaacgtacctttccatagcagctacgctcacagccaaagcctggaccgactaatgaatccactcatcgaccaatacttgtactatctctctagaactattaacggttctggacagaatcaacaaacgctaaaattcagtgtggccggacccagcaacatggctgtccagggaagaaactacatacctggacccagctaccgacaacaacgtgtctcaaccactgtgactcaaaacaacaacagcgaatttgcttggcctggagcttcttcttgggctctcaatggacgtaatagcttgatgaatcctggacctgctatggccagccacaaagaaggagaggaccgtttctttcctttgtctggatctttaatttttggcaaacaaggaactggaagagacaacgtggatgcggacaaagtcatgataaccaacgaagaagaaattaaaactactaacccggtagcaacggagtcctatggacaagtggccacaaaccaccagagtgcccaacaggcggttaggacgtctttggcacaggcgcagaccggttgggttcaaaaccaaggaatacttccgggtatggtttggcaggacagagatgtgtacctgcaaggacccatttgggccaaaattcctcacacggacggcaactttcacccttctccgctgatgggagggtttggaatgaagcacccgcctcctcagatcctcatcaaaaacacacctgtacctgcggatcctccaacggccttcaacaaggacaagctgaactctttcatcacccagtattctactggccaagtcagcgtggagatcgagtgggagctgcagaaggaaaacagcaagcgctggaacccggagatccagtacacttccaactattacaagtctaataatgttgaatttgctgttaatactgaaggtgtatatagtgaaccccgccccattggcaccagatacctgactcgtaatctgtaa

SEQ ID NO: 42 - DNA, 2229 bp, synthetic construct
  source 1..2229: mol_type = other DNA
atggctgccgatggttatcttccagattggctcgaggacaaccttagtgaaggaattcgcgagtggtgggctttgaaacctggagcccctcaacccaaggcaaatcaacaacatcaagacaacgctcgaggtcttgtgcttccgggttacaaataccttggacccggcaacggactcgacaagggggagccggtcaacgcagcagacgcggcggccctcgagcacgacaaggcctacgaccagcagctcaaggccggagacaacccgtacctcaagtacaaccacgccgacgccgagttccaggagcggctcaaagaagatacgtcttttgggggcaacctcgggcgagcagtcttccaggccaaaaagaggcttcttgaacctcttggtctggttgaggaagcggctaagacggctcctggaaagaagaggcctgtagagcagtctcctcaggaaccggactcctccgcgggtattggcaaatcgggtgcacagcccgctaaaaagagactcaatttcggtcagactggcgacacagagtcagtcccagaccctcaaccaatcggagaacctcccgcagccccctcaggtgtgggatctcttacaatggcttcaggtggtggcgcaccagtggcagacaataacgaaggtgccgatggagtgggtagttcctcgggaaattggcattgcgattcccaatggctgggggacagagtcatcaccaccagcacccgaacctgggccctgcccacctacaacaatcacctctacaagcaaatctccaacagcacatctggaggatcttcaaatgacaacgcctacttcggctacagcaccccctgggggtattttgacttcaacagattccactgccacttctcaccacgtgactggcagcgactcatcaacaacaactggggattccggcctaagcgactcaacttcaagctcttcaacattcaggtcaaagaggttacggacaacaatggagtcaagaccatcgccaataaccttaccagcacggtccaggtcttcacggactcagactatcagctcccgtacgtgctcgggtcggctcacgagggctgcctcccgccgttcccagcggacgttttcatgattcctcagtacgggtatctgacgcttaatgatggaagccaggccgtgggtcgttcgtccttttactgcctggaatatttcccgtcgcaaatgctaagaacgggtaacaacttccagttcagctacgagtttgagaacgtacctttccatagcagctacgctcacagccaaagcctggaccgactaatgaatccactcatcgaccaatacttgtactatctctctagaactattaacggttctggacagaatcaacaaacgctaaaattcagtgtggccggacccagcaacatggctgtccagggaagaaactacatacctggacccagctaccgacaacaacgtgtctcaaccactgtgactcaaaacaacaacagcgaatttgcttggcctggagcttcttcttgggctctcaatggacgtaatagcttgatgaatcctggacctgctatggccagccacaaagaaggagaggaccgtttctttcctttgtctggatctttaatttttggcaaacaaggtaccggcagagacaacgtggatgcggacaaagtcatgataaccaacgaagaagaaattaaaactactaacccggtagcaacggagtcctatggacaagtggccacaaaccaccagagtgcccaaactttggcggtgccttttaaggcacaggcgcagaccggttgggttcaaaaccaaggaatacttccgggtatggtttggcaggacagagatgtgtacctgcaaggacccatttgggccaaaattcctcacacggacggcaactttcacccttctccgctgatgggagggtttggaatgaagcacccgcctcctcagatcctcatcaaaaacacacctgtacctgcggatcctccaacggccttcaacaaggacaagctgaactctttcatcacccagtattctactggccaagtcagcgtggagatcgagtgggagctgcagaaggaaaacagcaagcgctggaacccggagatccagtacacttccaactattacaagtctaataatgttgaatttgctgttaatactgaaggtgtatatagtgaaccccgccccattggcaccagatacctgactcgtaatctg

SEQ ID NO: 43 - DNA, 1866 bp, Adeno-associated virus 2
  source 1..1866: mol_type = genomic DNA
atgccggggttttacgagattgtgattaaggtccccagcgaccttgacgagcatctgcccggcatttctgacagctttgtgaactgggtggccgagaaggaatgggagttgccgccagattctgacatggatctgaatctgattgagcaggcacccctgaccgtggccgagaagctgcagcgcgactttctgacggaatggcgccgtgtgagtaaggccccggaggcccttttctttgtgcaatttgagaagggagagagctacttccacatgcacgtgctcgtggaaaccaccggggtgaaatccatggttttgggacgtttcctgagtcagattcgcgaaaaactgattcagagaatttaccgcgggatcgagccgactttgccaaactggttcgcggtcacaaagaccagaaatggcgccggaggcgggaacaaggtggtggatgagtgctacatccccaattacttgctccccaaaacccagcctgagctccagtgggcgtggactaatatggaacagtatttaagcgcctgtttgaatctcacggagcgtaaacggttggtggcgcagcatctgacgcacgtgtcgcagacgcaggagcagaacaaagagaatcagaatcccaattctgatgcgccggtgatcagatcaaaaacttcagccaggtacatggagctggtcgggtggctcgtggacaaggggattacctcggagaagcagtggatccaggaggaccaggcctcatacatctccttcaatgcggcctccaactcgcggtcccaaatcaaggctgccttggacaatgcgggaaagattatgagcctgactaaaaccgcccccgactacctggtgggccagcagcccgtggaggacatttccagcaatcggatttataaaattttggaactaaacgggtacgatccccaatatgcggcttccgtctttctgggatgggccacgaaaaagttcggcaagaggaacaccatctggctgtttgggcctgcaactaccgggaagaccaacatcgcggaggccatagcccacactgtgcccttctacgggtgcgtaaactggaccaatgagaactttcccttcaacgactgtgtcgacaagatggtgatctggtgggaggaggggaagatgaccgccaaggtcgtggagtcggccaaagccattctcggaggaagcaaggtgcgcgtggaccagaaatgcaagtcctcggcccagatagacccgactcccgtgatcgtcacctccaacaccaacatgtgcgccgtgattgacgggaactcaacgaccttcgaacaccagcagccgttgcaagaccggatgttcaaatttgaactcacccgccgtctggatcatgactttgggaaggtcaccaagcaggaagtcaaagactttttccggtgggcaaaggatcacgtggttgaggtggagcatgaattctacgtcaaaaagggtggagccaagaaaagacccgcccccagtgacgcagatataagtgagcccaaacgggtgcgcgagtcagttgcgcagccatcgacgtcagacgcggaagcttcgatcaactacgcagacaggtaccaaaacaaatgttctcgtcacgtgggcatgaatctgatgctgtttccctgcagacaatgcgagagaatgaatcagaattcaaatatctgcttcactcacggacagaaagactgtttagagtgctttcccgtgtcagaatctcaacccgtttctgtcgtcaaaaaggcgtatcagaaactgtgctacattcatcatatcatgggaaaggtgccagacgcttgcactgcctgcgatctggtcaatgtggatttggatgactgcatctttgaacaataa

SEQ ID NO: 44 - DNA, 1866 bp, Adeno-associated virus
  source 1..1866: mol_type = genomic DNA
atgccggggttttacgagattgtgattaaggtccccagcgaccttgacgagcatctgcccggcatttctgacagctttgtgaactgggtggccgagaaggaatgggagttgccgccagattctgacatggatctgaatctgattgagcaggcacccctgaccgtggccgagaagctgcagcgcgactttctgacggaatggcgccgtgtgagtaaggccccggaggctcttttctttgtgcaatttgagaagggagagagctacttccacatgcacgtgctcgtggaaaccaccggggtgaaatccatggttttgggacgtttcctgagtcagattcgcgaaaaactgattcagagaatttaccgcgggatcgagccgactttgccaaactggttcgcggtcacaaagaccagaaatggcgccggaggcgggaacaaggtggtggatgagtgctacatccccaattacttgctccccaaaacccagcctgagctccagtgggcgtggactaatatggaacagtatttaagcgcctgtttgaatctcacggagcgtaaacggttggtggcgcagcatctgacgcacgtgtcgcagacgcaggagcagaacaaagagaatcagaatcccaattctgatgcgccggtgatcagatcaaaaacttcagccaggtacatggagctggtcgggtggctcgtggacaaggggattacctcggagaagcagtggatccaggaggaccaggcctcatacatctccttcaatgcggcctccaactcgcggtcccaaatcaaggctgccttggacaatgcgggaaagattatgagcctgactaaaaccgcccccgactacctggtgggccagcagcccgtggaggacatttccagcaatcggatttataaaattttggaactaaacgggtacgatccccaatatgcggcttccgtctttctgggatgggccacgaaaaagttcggcaagaggaacaccatctggctgtttgggcctgcaactaccgggaagaccaacatcgcggaggccatagcccacactgtgcccttctacgggtgcgtaaactggaccaatgagaactttcccttcaacgactgtgtggacaagatggtgatctggtgggaggaggggaagatgaccgccaaggtcgtggagtcggccaaagccattctcggaggaagcaaggtgcgcgtggaccagaaatgcaagtcctcggcccagatagacccgactcccgtgatcgtcacctccaacaccaatatgtgcgccgtgattgacgggaactcaacgaccttcgaacaccagcagccgttgcaagaccggatgttcaaatttgaactcacccgccgtctggatcatgactttgggaaggtcaccaagcaggaagtcaaagactttttccggtgggcaaaggatcacgtggttgaggtggagcatgaattctacgtcaaaaagggtggagccaagaaaagacccgcccccagtgacgcagatataagtgagcccaaacgggtgcgcgagtcagttgcgcagccatcgacgtcagacgcggaagcttcgatcaactacgcggacaggtaccaaaacaaatgttctcgtcacgtgggcatgaatctgatgctgtttccctgcagacaatgcgagagactgaatcagaattcaaatatctgcttcactcacggtgtcaaagactgtttagagtgctttcccgtgtcagaatctcaacccgtttctgtcgtcaaaaaggcgtatcagaaactgtgctacattcatcacatcatgggaaaggtgccagacgcttgcactgcttgcgacctggtcaatgtggacttggatgactgtgtttctgaacaataa

SEQ ID NO: 45 - protein, 621 aa, Adeno-associated virus 2
MPGFYEIVIKVPSDLDEHLPGISDSFVNWVAEKEWELPPDSDMDLNLIEQAPLTVAEKLQRDFLTEWRRVSKAPEALFFVQFEKGESYFHMHVLVETTGVKSMVLGRFLSQIREKLIQRIYRGIEPTLPNWFAVTKTRNGAGGGNKVVDECYIPNYLLPKTQPELQWAWTNMEQYLSACLNLTERKRLVAQHLTHVSQTQEQNKENQNPNSDAPVIRSKTSARYMELVGWLVDKGITSEKQWIQEDQASYISFNAASNSRSQIKAALDNAGKIMSLTKTAPDYLVGQQPVEDISSNRIYKILELNGYDPQYAASVFLGWATKKFGKRNTIWLFGPATTGKTNIAEAIAHTVPFYGCVNWTNENFPFNDCVDKMVIWWEEGKMTAKVVESAKAILGGSKVRVDQKCKSSAQIDPTPVIVTSNTNMCAVIDGNSTTFEHQQPLQDRMFKFELTRRLDHDFGKVTKQEVKDFFRWAKDHVVEVEHEFYVKKGGAKKRPAPSDADISEPKRVRESVAQPSTSDAEASINYADRYQNKCSRHVGMNLMLFPCRQCERMNQNSNICFTHGQKDCLECFPVSESQPVSVVKKAYQKLCYIHHIMGKVPDACTACDLVNVDLDDCIFEQ

SEQ ID NO: 46 - protein, 621 aa, Adeno-associated virus
MPGFYEIVIKVPSDLDEHLPGISDSFVNWVAEKEWELPPDSDMDLNLIEQAPLTVAEKLQRDFLTEWRRVSKAPEALFFVQFEKGESYFHMHVLVETTGVKSMVLGRFLSQIREKLIQRIYRGIEPTLPNWFAVTKTRNGAGGGNKVVDECYIPNYLLPKTQPELQWAWTNMEQYLSACLNLTERKRLVAQHLTHVSQTQEQNKENQNPNSDAPVIRSKTSARYMELVGWLVDKGITSEKQWIQEDQASYISFNAASNSRSQIKAALDNAGKIMSLTKTAPDYLVGQQPVEDISSNRIYKILELNGYDPQYAASVFLGWATKKFGKRNTIWLFGPATTGKTNIAEAIAHTVPFYGCVNWTNENFPFNDCVDKMVIWWEEGKMTAKVVESAKAILGGSKVRVDQKCKSSAQIDPTPVIVTSNTNMCAVIDGNSTTFEHQQPLQDRMFKFELTRRLDHDFGKVTKQEVKDFFRWAKDHVVEVEHEFYVKKGGAKKRPAPSDADISEPKRVRESVAQPSTSDAEASINYADRYQNKCSRHVGMNLMLFPCRQCERLNQNSNICFTHGVKDCLECFPVSESQPVSVVKKAYQKLCYIHHIMGKVPDACTACDLVNVDLDDCVSEQ

SEQ ID NO: 47 - DNA, 131 bp, synthetic construct
  source 1..131: mol_type = other DNA
gtttatttgtgaaatttgtgatgctattgctttatttgtaaccattataagctgcaataaacaagttaacaacaacaattgcattcattttatgtttcaggttcagggggagatgtgggaggttttttaaa

SEQ ID NO: 48 - DNA, 7326 bp, synthetic construct
  source 1..7326: mol_type = other DNA
gcgcgccgatatcgttaacgccccgcgccggccgctctagaactagtggatcccccggaagatcagaagttcctattccgaagttcctattctctagaaagtataggaacttctgatctgcgcagccgccatgccggggttttacgagattgtgattaaggtccccagcgaccttgacgagcatctgcccggcatttctgacagctttgtgaactgggtggccgagaaggaatgggagttgccgccagattctgacatggatctgaatctgattgagcaggcacccctgaccgtggccgagaagctgcagcgcgactttctgacggaatggcgccgtgtgagtaaggccccggaggcccttttctttgtgcaatttgagaagggagagagctacttccacatgcacgtgctcgtggaaaccaccggggtgaaatccatggttttgggacgtttcctgagtcagattcgcgaaaaactgattcagagaatttaccgcgggatcgagccgactttgccaaactggttcgcggtcacaaagaccagaaatggcgccggaggcgggaacaaggtggtggatgagtgctacatccccaattacttgctccccaaaacccagcctgagctccagtgggcgtggactaatatggaacagtatttaagcgcctgtttgaatctcacggagcgtaaacggttggtggcgcagcatctgacgcacgtgtcgcagacgcaggagcagaacaaagagaatcagaatcccaattctgatgcgccggtgatcagatcaaaaacttcagccaggtacatggagctggtcgggtggctcgtggacaaggggattacctcggagaagcagtggatccaggaggaccaggcctcatacatctccttcaatgcggcctccaactcgcggtcccaaatcaaggctgccttggacaatgcgggaaagattatgagcctgactaaaaccgcccccgactacctggtgggccagcagcccgtggaggacatttccagcaatcggatttataaaattttggaactaaacgggtacgatccccaatatgcggcttccgtctttctgggatgggccacgaaaaagttcggcaagaggaacaccatctggctgtttgggcctgcaactaccgggaagaccaacatcgcggaggccatagcccacactgtgcccttctacgggtgcgtaaactggaccaatgagaactttcccttcaacgactgtgtcgacaagatggtgatctggtgggaggaggggaagatgaccgccaaggtcgtggagtcggccaaagccattctcggaggaagcaaggtgcgcgtggaccagaaatgcaagtcctcggcccagatagacccgactcccgtgatcgtcacctccaacaccaacatgtgcgccgtgattgacgggaactcaacgaccttcgaacaccagcagccgttgcaagaccggatgttcaaatttgaactcacccgccgtctggatcatgactttgggaaggtcaccaagcaggaagtcaaagactttttccggtgggcaaaggatcacgtggttgaggtggagcatgaattctacgtcaaaaagggtggagccaagaaaagacccgcccccagtgacgcagatataagtgagcccaaacgggtgcgcgagtcagttgcgcagccatcgacgtcagacgcggaagcttcgatcaactacgcagacaggtaccaaaacaaatgttctcgtcacgtgggcatgaatctgatgctgtttccctgcagacaatgcgagagaatgaatcagaattcaaatatctgcttcactcacggacagaaagactgtttagagtgctttcccgtgtcagaatctcaacccgtttctgtcgtcaaaaaggcgtatcagaaactgtgctacattcatcatatcatgggaaaggtgccagacgcttgcactgcctgcgatctggtcaatgtggatttggatgactgcatctttgaacaataaatgatttaaatcaggtatggctgccgatggttatcttccagattggctcgaggacactctctctgaaggaataagacagtggtggaagctcaaacctggcccaccaccaccaaagcccgcagagcggcataaggacgacagcaggggtcttgtgcttcctgggtacaagtacctcggacccttcaacggactcgacaagggagagccggtcaacgaggcagacgccgcggccctcgagcacgacaaagcctacgaccggcagctcgacagcggagacaacccgtacctcaagtacaaccacgccgacgcggagtttcaggagcgccttaaagaagatacgtcttttgggggcaacctcggacgagcagtcttccaggcgaaaaagagggttcttgaacctctgggcctggttgaggaacctgttaagacggctccgggaaaaaagaggccggtagagcactctcctgtggagccagactcctcctcgggaaccggaaaggcgggccagcagcctgcaagaaaaagattgaattttggtcagactggagacgcagactcagtacctgacccccagcctctcggacagccaccagcagccccctctggtctgggaactaatacgatggctacaggcagtggcgcaccaatggcagacaataacgagggcgccgacggagtgggtaattcctcgggaaattggcattgcgattccacatggatgggcgacagagtcatcaccaccagcacccgaacctgggccctgcccacctacaacaaccacctctacaaacaaatttccagccaatcaggagcctcgaacgacaatcactactttggctacagcaccccttgggggtattttgacttcaacagattccactgccacttttcaccacgtgactggcaaagactcatcaacaacaactggggattccgacccaagagactcaacttcaagctctttaacattcaagtcaaagaggtcacgcagaatgacggtacgacgacgattgccaataaccttaccagcacggttcaggtgtttactgactcggagtaccagctcccgtacgtcctcggctcggcgcatcaaggatgcctcccgccgttcccagcagacgtcttcatggtgccacagtatggatacctcaccctgaacaacgggagtcaggcagtaggacgctcttcattttactgcctggagtactttccttctcagatgctgcgtaccggaaacaactttaccttcagctacacttttgaggacgttcctttccacagcagctacgctcacagccagagtctggaccgtctcatgaatcctctcatcgaccagtacctgtattacttgagcagaacaaacactccaagtggaaccaccacgcagtcaaggcttcagttttctcaggccggagcgagtgacattcgggaccagtctaggaactggcttcctggaccctgttaccgccagcagcgagtatcaaagacatctgcggataacaacaacagtgaatactcgtggactggagctaccaagtaccacctcaatggcagagactctctggtgaatccgggcccggccatggcaagccacaaggacgatgaagaaaagttttttcctcagagcggggttctcatctttgggaagcaaggctcagagaaaacaaatgtggacattgaaaaggtcatgattacagacgaagaggaaatcaggacaaccaatcccgtggctacggagcagtatggttctgtatctaccaacctccagagaggcaacagacaagcagctaccgcagatgtcaacacacaaggcgttcttccaggcatggtctggcaggacagagatgtgtaccttcaggggcccatctgggcaaagattccacacacggacggacattttcacccctctcccctcatgggtggattcggacttaaacaccctcctccacagattctcatcaagaacaccccggtacctgcgaatccttcgaccaccttcagtgcggcaaagtttgcttccttcatcacacagtactccacgggacaggtcagcgtggagatcgagtgggagctgcagaaggaaaacagcaaacgctggaatcccgaaattcagtacacttccaactacaacaagtctgttaatgtggactttactgtggacactaatggcgtgtattcagagcctcgccccattggcaccagatacctgactcgtaatctgtaattgcttgttaatcaataaaccgtttaattcgtttcagttgaactttggtctctgcgtatttctttcttatctagtttccatggctacgtagataagtagcatggcgggttaatcattaactacagcccgggcgtttaaacagcgggcggaggggtggagtcgtgacgtgaattacgtcatagggttagggaggtcctgtattagaggtcacgtgagtgttttgcgacattttgcgacaccatgtggtctcgctgggggggggggcccgagtgagcacgcagggtctccattttgaagcgggaggtttgaacgagcgctggcgcgctcactggccgtcgttttacaacgtcgtgactgggaaaaccctggcgttacccaacttaatcgccttgcagcacatccccctttcgccagctggcgtaatagcgaagaggcccgcaccgatcgcccttcccaacagttgcgcagcctgaatggcgaatggaaattgtaagcgttaatattttgttaaaattcgcgttaaatttttgttaaatcagctcatttttttaaccaataggccgaaatcggcaaaatcccttataaatcaaaagaatagaccgagatagggttgagtgttgttccagtttggaacaagagtccactattaagaacgtggactccaacgtcaaagggcgaaaaaccgtctatcagggcgatggcccactacgtgaaccatcaccctaatcaagttttttggggtcgaggtgccgtaaagcactaaatcggaaccctaaagggagcccccgatttagagcttgacggggaaagccggcgaacgtggcgagaaaggaagggaagaaagcgaaaggagcgggcgctagggcgctggcaagtgtagcggtcacgctgcgcgtaaccaccacacccgccgcgcttaatgcgccgctacagggcgcgtcaggtggcacttttcggggaaatgtgcgcggaacccctatttgtttatttttctaaatacattcaaatatgtatccgctcatgagacaataaccctgataaatgcttcaataatattgaaaaaggaagagtatgagtattcaacatttccgtgtcgcccttattcccttttttgcggcattttgccttcctgtttttgctcacccagaaacgctggtgaaagtaaaagatgctgaagatcagttgggtgcacgagtgggttacatcgaactggatctcaacagcggtaagatccttgagagttttcgccccgaagaacgttttccaatgatgagcacttttaaagttctgctatgtggcgcggtattatcccgtattgacgccgggcaagagcaactcggtcgccgcatacactattctcagaatgacttggttgagtactcaccagtcacagaaaagcatcttacggatggcatgacagtaagagaattatgcagtgctgccataaccatgagtgataacactgcggccaacttacttctgacaacgatcggaggaccgaaggagctaaccgcttttttgcacaacatgggggatcatgtaactcgccttgatcgttgggaaccggagctgaatgaagccataccaaacgacgagcgtgacaccacgatgcctgtagcaatggcaacaacgttgcgcaaactattaactggcgaactacttactctagcttcccggcaacaattaatagactggatggaggcggataaagttgcaggaccacttctgcgctcggcccttccggctggctggtttattgctgataaatctggagccggtgagcgtgggtctcgcggtatcattgcagcactggggccagatggtaagcctcccgtatcgtagttatctacacgacggggagtcaggcaactatggatgaacgaaatagacagatcgctgagataggtgcctcactgattaagcattggtaactgtcagaccaagtttactcatatatactttagattgatttaaaacttcatttttaatttaaaaggatctaggtgaagatcctttttgataatctcatgaccaaaatcccttaacgtgagttttcgttccactgagcgtcagaccccgtagaaaagatcaaaggatcttcttgagatcctttttttctgcgcgtaatctgctgcttgcaaacaaaaaaaccaccgctaccagcggtggtttgtttgccggatcaagagctaccaactctttttccgaaggtaactggcttcagcagagcgcagataccaaatactgttcttctagtgtagccgtagttaggccaccacttcaagaactctgtagcaccgcctacatacctcgctctgctaatcctgttaccagtggctgctgccagtggcgataagtcgtgtcttaccgggttggactcaagacgatagttaccggataaggcgcagcggtcgggctgaacggggggttcgtgcacacagcccagcttggagcgaacgacctacaccgaactgagatacctacagcgtgagctatgagaaagcgccacgcttcccgaagggagaaaggcggacaggtatccggtaagcggcagggtcggaacaggagagcgcacgagggagcttccagggggaaacgcctggtatctttatagtcctgtcgggtttcgccacctctgacttgagcgtcgatttttgtgatgctcgtcaggggggcggagcctatggaaaaacgccagcaacgcggcctttttacggttcctggccttttgctggccttttgctcacatgttctttcctgcgttatcccctgattctgtggataaccgtattaccgcctttgagtgagctgataccgctcgccgcagccgaacgaccgagcgcagcgagtcagtgagcgaggaagcggaagagcgcccaatacgcaaaccgcctctccccgcgcgttggccgattcattaatgcagctggcacgacaggtttcccgactggaaagcgggcagtgagcgcaacgcaattaatgtgagttagctcactcattaggcaccccaggctttacactttatgcttccggctcgtatgttgtgtggaattgtgagcggataacaatttcacacaggaaacagctatgaccatgattacgccaa